European Patent Specification EP 3 622 076 B1, published April 16, 2025. Title: Insecticidal Proteins and Methods for Their Use. Applicant: Pioneer Hi-Bred International, Inc. The sequence listing filed with the application follows.

SEQUENCE LISTING (249 sequences)

SEQ ID NO: 1 - DNA, 637 bp, Polystichum tripteron
atgggcaggtcatggggagttgtggctattatggtgttgtgcgccagcggcctgctgggcgtagcgagcggccatggcaccatgaacgaccccatcagtcgcgtctacgcctgcaggcaggagaatccggagcgacccactacgccggcttgcatagcggcggtggcgctgagtggggcccaagcgttctatgattggaatgaggtgaacctgccctttgtcaatggccggcaccgccagttcattccggatgggaaactctgcagcgccgggcggaacaagtataggggtctcgacctggcacgctccgactggacagccacaaacttgtcctccggcgtcgcctacacattcctctacagggtcaccgcccagcacaggggcttcttcgagttctacgtcaccgtggatggttacgaccccactgagccgctcaaatgggcagacttggaggaaacgccgttcatcaacgtcaccgaccccacagttgtaggcctcaactatgtaatccccggtaccacgcctgccagcaagaccggccgccacctcatctacgtcatttggcagcgctccgacagccccgaggccttctactcctgctccgacgtcaactttcccgatgccctgtctctccact

SEQ ID NO: 2 - DNA, 637 bp, Polystichum tripteron
atgggcaggtcatggggagttgtggctattatggtgttgtgcgccagcggcctgctgggcgtagcgagcggccatggcaccatgaacgaccccatcagtcgcgtctacgcctgcaggcaggagaatccggagcgacccactacgccggcttgcatagcggcggtggcgctgagtggggcccaagcgttctatgattggaatgaggtgaacattcctaatgcccctggtcggcaccgtgagctcatttctgatggctacctatgcagcgccaatcggaccaagtatgcaggtctcgacctggcacgctccgactggacagccacaaacttgtcctccggcgtcgcctacacattcctctacagggtcaccgcccagcacaggggcttcttcgagttctacgtcaccgtggatggttacgaccccactgagccgctcaaatgggcagacttggaggaaacgccgttcatcaacgtcaccgaccccacagttgtaggcctcaactatgtaatccccggtaccacgcctgccagcaagaccggccgccacctcatctacgtcatttggcagcgctccgacagccccgaggccttctactcctgctccgacgtcaactttcccgatgccctgtctctccact

SEQ ID NO: 3 - DNA, 643 bp, Davallia fejeensis
atgggcaggtcatggggagttgttgcaattatggtggtgtgcatcatgagtggcctggtgggcatagtgagtggccatggcagcatggaggaccccatcagtcgcgtctatagatgctacttagagaatccggagcgtcctgtatcggcagcttgccaagcagcggtggcgatgagtggtacccaagccttctacgattggaatgaggtgaacattcctaacgccgctggccggcaccgtgagctcatttccgatggccaactatgcagcgccaatcgcacaaagtatgcaggccttgacttggcacgcgctgactggctaggcacccccttgtcctcgggtgtctccttcacatttgcctacaaggccaccgcaccacacttgggctttttcgagttctacgttacccgggatggttacgagcccaccgagccgctcaaatgggcggacttagaggactcgccctttatcaatgtcaccgaccccacacttgaaaatggcgcctaccaaatctctggcactacaccttctggtaagtcggggcgccacttgatgtatgtcatttggcagcgctctgatagccctgaggcgttctactcgtgctccgatgttgacttcgacgtcgatgccctctctctccact

SEQ ID NO: 4 - DNA, 635 bp, Didymochlaena truncatula
atgggcaggtcatggggagttgtggctattatggtgttgtgcgccagcggcctgctgggcgtagcgagtggccatggcagcatggaggaccctatcagtcgcgtctacgcctgctacctggagaatccggagcgtcccacgtcggcagcttgccaagcggcggtggcagtgagtgggacccaagcgttctatgattggaatgaggtgaaccagcccttcgccgctggccggcaccgcgagctcattccggatggcgaactgtgcagcggcgggcgggagaagtataagggcctcgacttggcacgcgccgactggccagccacctccttgccctccggtgtcaactacacatacctctacaaggccaccgccccgcacttgggcttcttcgagttctacatcacccgggatggctacgagcccactgagccgctcaaatgggcagacttggaggacttgccgttcatcaacatcaccaaccccacgcttgtcagcggctcctaccaaatccccggcaccacgcatgccagcaagactggccggcacctcctctatgtcatttggcagcgctccgacagcttcgaggccttctactcctgctccgacgtcgacttcgtcaatgccctctctctcca

SEQ ID NO: 5 - DNA, 636 bp, Didymochlaena truncatula
atgggcaggtcatggggagttgtggctattatggtgttgtgcgccagcggcctgctgggcgtagcgagtggccatggcagcatggaggaccctatcagtcgcgtctacgcctgctacctggagaatccggagcgtcccacgtcggcagcttgccaagcggcggtggcagtgagtgggacccaagcgttctatgattggaatgaggtgaaccagcccttcgccgctggccggcaccgcgagctcattccggatggcgaactgtgcagcggcgggcgggagaagtataagggcctcgacttggcacgcgccgactggccagccacctccttgccctccggtgtcaactacacatacctctacaaggccaccgccccgcacttgggcttcttcgagttctacatcacccgggatggctacgagcccactgagccgctcaaatgggcagacttggaggacttgccgttcatcaacatcaccaaccccacgcttgtcagcggctcctaccaaatccccggcaccacgcctgccagcaagactggccggcacctcctctatgtcatttggcagcgctccgacagcttcgaggccttctactcctgctccgacgtcgacttcgtcaatgccctctctctccac

SEQ ID NO: 6 - DNA, 636 bp, Humata tyermanii
atgggcaggtcatggggagttgtggctattatggtgatgtacattggtggcctgctaagcatagcaagcggccatggcagcatggaggaccccatcagccgcgtctataggtgctacttggagaatccggagagtcccacatcggcagcttgccaagcggcagtggcagtgagtggggcccaagccttctacgattggaatgaggtgaacattgctgacgccaatggccgacaccgggagctcatttctgatggccaactatgtagcgcaaatcggagtaagtatgcgggcctcgacctggcacgcgcagattggctaggcaccaccttgtcctcgggcgcctccttcacatttgcctacaaggccaccgcgccgcacttgggcttctttgagttctacgtcacccgggatggttacgagcccaccgacccgctcaaatgggcagacttggaggactcgcccttcatcaacgtcaccaaccccacacttgataatggcgcctaccagatctccggcaccacgcctgccggtaagtcggggcgtcatctgatctacgtcatttggcagcgctctgatagcccagaggcattctattcgtgctccgacgtcgactttgtcgatgctctctctctccac

SEQ ID NO: 7 - DNA, 726 bp, Cyrtomium fortunei
atggggagttgtggctattatggtgttgtgcgccagcggcctgctgggcgtggcggcaattctgttggtcatagtgtggggatggggaggtcatggggagttgtggctattatggtgctgtgcaccagcggcctgctgggcgtggcgagcggccatggcaccatgggcgaccccatcagccgcgtctacaactgcttccaggagaatccggagagacccacgtcggcagcttgcatcgcggcggtggcgctcagtggaacccaagcgttctatgattggaatgaggtgaacctgcccgacgtcaatggccgccaccgcgagttcattccggatggccaactgtgcagcgccgggcgggacaagtataagggtctcgacctggcacgctccgactggacagccaccaacttgtcctccggcgtcgcctacacattcctctacagggtcaccgcccagcacaggggcttcttcgagttctacgtcaccgtggatgattacgatcccactgtggcgctcaaatgggaggacttggaggaaacaccgttcctcaacgtcaccgaccccacggttgtaggcgtcaactaccaaatctccggcaccacgcctgccagcaagaccggccgccacctcatctacgtcatttggcagcgctccgacagccctgaggccttctacgcctgctccgatgtcgacttcgtcgatgccgtctctctccactccaccacc

SEQ ID NO: 8 - DNA, 741 bp, Adiantum hispidulum
atgaagaagtcatggggacttgcagtagtagtaggttcacatctgattgtaaggatgaagaagtcatggggagttgcagtagtagtaggagtagtagctttgtgcctgctgggcatggcaagcggccatggcagcatgcaggaccccatcagtcgcgtctacaactgctacctagagggcccggagcgcccaacgtcggcagcttgcatagctgcggtggcaatgagtggcacacaaccattctacgattggaatgaggtgaacttgcccgacgccgctggccggcaccgcgagctcatccccgatggcaagctgtgcagcgccggccgggataagtatcagggcctcgacctggcgcgcgacgactgggtagcctccttatcctctggcgtcgcctacacattcctttaccgagtcactgcccagcacttgggcttctttgaaatttacgtcacccgtgacacctacgaccccactcaggcgctaacatgggatgacctggaagactcgcccttcatcaacgttaccaacccctccgttgtcagtacgacgttgggtaacgcctacgcaatccccacccccacgccatccggcaagactggtcgccacctcatctacgtaatctggcagcgcagcgacagccccgaggcgttctactcctgctccgacgtcgagttcgacgtggcatcgacagtcgaggacgacgtcatcatctctctccgctccgcagctctagacgtc

SEQ ID NO: 9 - DNA, 750 bp, Polystichum acrostichoides
atggtcacctatatatatatgtgtgaaatgcatgttggaaggtgtagcaatatgcgtgcagtaattagagaagccaattatattgatcatagtgtgagtgtgagcatggggaggtcatggggagttgtggctattatggtgttgtgcgctagcggcctgctgggtgtagcgagcggccatggcagcatgaacgaccccatcagccgcgtctacaactgccgtctggagaatccggagagtcccacgtcagcagcttgcatagcggcggtggcgctgagtgggacccaagcgttctatgattggaatgaggtgaacctgcccgacgtcaatggccggcaccgccagctcattccggatggcaaattgtgcagcgccgggcgggacaagtataagggcctcgacctggcacgctccgactgggtagccaccaacttgtcctccggcgtcgccttcacattcctctacagggtcaccgcccagcacaggggcttcttcgagttctacgtcaccgtggatgattacgaccccactgagctgctcaaatgggaagacttggaggaaacgccgttcatgaacgtcaccgaccccacggttgtaggcgtcaactacgaaatccccggcaccacgcctgccaataagaccggccgccatctcatctatgtcatttggcagcgctccgacagccccgaggccttctactcctgctccgacgttgacttcgtcgatgccgtgtctctccactccaccacc

SEQ ID NO: 10 - DNA, 729 bp, Thelypteris kunthii
atgcatgttggaatatacagcacgagtgcagtagtagggaggatgagagaaagcaatattggtcataacaccgtgaggatggagagggctgcatggggcgttgtgggcattattatggtgttgtgcgccagcggcctgctgggcgtagcgagtggccacggcagcatggaggaccccatcagtcgcgtctacctctgctacctcgagaatccggagcgtcccacgtcggcagcttgccaagcggcggtggcgctgagtgggacccaagcattctatgattggaatgaggtgaacatcgccgacgccgctggccggcaccgcgagctcattccggatggccaactgtgcagcgccgggcgggacaagtataagggcctcgacctggcacgctccgactgggtagccaccaacttgtcctccggcgtcgccttcacattcctctacagggtcaccgccgagcacaggggcttcttcgagttctacgtcaccgtggatgattacgaccccactgagctgctcaaatgggaagacttggaggcaacgccgttcatgaatgtcaccgaccccacggttgtaggcgacaactacgaaatccccggcaccacgcctgccaacaagaccggccgccatctcatctatgtcatttggcagcgctccgacagccccgaggccttctactcctgctctgacgtcgtcttcgccgatgccgtgtctctccactccaccacc

SEQ ID NO: 11 - DNA, 747 bp, Cyrtomium fortune (clivicola)
atgcattctggaatgggcagcagtatgcgtgcagcaattaggaggacgagacaaggcaattatactggtcatagtgtgaggatggggacattggggaggtcatggggagctgtggctattatggtgttgtgcgccagcggtctcctgggcgtagccagcggccatggcagcatgaacgaccccatcagccgcgtctacaactgctacctggagaatccggagagacccacctcggcagcttgcatagcggccgtggcgctcagtgggacccaagcgttctatgattggaatgaggtgaatctgcccgacgccaatggccggcaccgccagctcattccggatggccaactgtgcagcgccgggcgggacaagtataaaggcctcgacctcgcacgctccgactggacggccaccaatttatcctccggcgtcgccttcacattcctctacagggtcaccgcccagcacaggggcttcttcgagttctacgtcaccgtggatgattacgatcccactgtggcgctcaaatgggaggacttggaggaaacaccgttcctcaacgtcaccgaccccacggttgtaggcgtcaactaccaaatctccggcaccacgcctgccagcaagaccggccgccacctcatctacgtcatttggcagcgctccgacagccccgaggctttctatgcctgctccgacgtcgactttgtcgatgccgtctctctccactccaccaccttgaccctgatc

SEQ ID NO: 12 - DNA, 729 bp, Polystichum tripteron
atgcatgttggaatgtgcagcaatatgcttgcagtaattaggaggacgagacatttaggcacttattttggtcatagtgtgaggatgggcaggtcatggggagttgtggctattatggtgttgttttccagtggcctgctgggagtagcaagcggccatggcagcatgggcgaccccatcagtcgcgtctacaactgcaggcaggagaatccggagcgacccactacgccggcttgcatagcggcggtggcgctgagtggggcccaagcgttctatgattggaatgaggtgaacctgccctttgtcaatggccggcaccgccagttcattccggatgggaaactctgcagcgccgggcggaacaagtataggggtctcgacctggcacgctccgactggacagccacaaacttgtcctccggcgtcgcctacacattcctctacagggtcaccgcccagcacaggggcttcttcgagttctacgtcaccgtggatggttacgaccccactgagccgctcaaatgggcagacttggaggaaacgccgttcatcaacgtcaccgaccccacagtagaaggcctcaactatgttcgagttctacgtcaccgtggatgcaagagtggccgccacctcatctacgtcatttggcagcgctccgacagccccgaggccttctactcctgctccgacgtcaactttcccgatgccctgtctctccactccgccacc

SEQ ID NO: 13 - DNA, 744 bp, Didymochlaena truncatula
atgatcacctgtatatatatgtgtgaaatgcatgttgaaatgtgcaacatgcgtgcagtagggaggctgagacaaggcaatattggtcatagtgtgaggatggggagatcatggggagttgtggctattatggtgttgtgcgccagcggcctgctgggcgtagcgagtggccatggcagcatggaggaccctatcagtcgcgtctacgcctgctacctggagaatccggagcgtcccacgtcggcagcttgccaagcggcggtggcagtgagtgggacccaagcgttctatgattggaatgaggtgaaccagcccttcgccgctggccggcaccgcgagctcattccggatggcgaactgtgcagcggcgggcgggagaagtataagggcctcgacttggcacgcgccgactggccagccacctccttgccctccggtgtcaactacacatacctctacaaggccaccgccccgcacttgggcttcttcgagttctacatcacccgggatggctacgagcccactgagccgctcaaatgggcagacttggaggacttgccgttcatcaacatcaccaaccccacgcttgtcagcggctcctaccaaatccccggcaccacgcctgccagcaagactggccggcacctcctctatgtcatttggcagcgctccgacagcttcgaggccttctactcctgctccgacgtcgacttcgtcaatgccctctctctccactccaccacc

SEQ ID NO: 14 - DNA, 750 bp, Asplenium antiquum
atgtcgagacgctggctgtcattcaatcacacaaacattgggttgcattttttgagtagtgctatgagaatggggaggtcggcatcttgcatcagagctaatatggcgatcatgctggtgttgttttgggctagctgctcctgcctgctgggcatagtgagcgggcatggcagcatggaggatcccatcagtcgtgtctacgcctgcttcttggagaatccggagaggcccacatctgcagcttgcatagcggcggtggcgttgagtgggacgcaagcgttctacgattggaacgaggttaaccagcccaacgccgccggtcggcaccgcgagatcattccggatggccagctttgcggcgccggacgggacaagtataagggcctcaacttggcacgtgccgactggccggcaaccaccttgtcctccgacatcagcttcacatacctcttcaaggcaaccgcccctcaccgcggtttcttcgagttctacgtcacccgggatggttacgatcccaccgagcccctcaaatgggcggacttggaggacccaccattcctcaacgtcaccgaccccacgcttgcttccggctcctaccaaatccccggcaccacaccagccggcaagactggccgccatctcatttacgtcatatggcagcgctccgatagccccgaagccttctactcttgctctgacgtggactttgacagcagcgataccgtgatctctctccgctctgccaccacc

SEQ ID NO: 15 - DNA, 720 bp, Cyrtomium falcatum (Butterfieldii)
atgttggaatgtgcagcaaatatgcgtgcagtaattagcaggacgagacaaggcaattctattgtgagtgtgaggatggggaggtcatggggagttgtggctattatggtgttgtgcgccaccggcctcctgggcgtggcgagcggccatggcagcatgggcgaccccatcagccgcgtctacaactgcttcctggagaatcctgagagacccacgtcggcagcttgcatcgcggccgttgcgctcagtggaacccaagcgttctatgattggaatgaggtgaacctgcccgacgtcaatggccgccaccgccagttcattccggatggccaactgtgcagcgccgggcgggacaagtataagggtctcgacctggcacgctccgactggacagccaccaacttgtcctccggcatcgcctacacattcctctacagggtcaccgcccagcacaggggcttcttcgagttctacgtcaccgtggatgattacgatcccactgtggcgctcaaatgggaggacttggaggaaacgccgttcctcaacgtcaccgaccccacggttgtaggcgtcaactaccagatcaacggcaccacgcctgccagcaagacgggccgccacctcatctacgtcatttggcagcgctccgacagccccgaggccttctacgcctgctccgacgtcgacttcgtcgatgccgtctctctccactccaccacc

SEQ ID NO: 16 - DNA, 741 bp, Onoclea sensibilis
atgcgtgcagtcattagtaagaagatattgagacaaggcaatattggtgatattggtgatagtgtgatcactgattcagccttgaggatggggaggtcatggggagtggtgcaggctataattatggtgttgtgcggcagcggcctgctgggcgtagcgagcggccatggcagcatggaggaccccatcagtcgcgtctacaactgctacctggagaatcccgagagtcccacgtcggcagcttgccaagcggcggtggcgctgagtggggcccaagcgttctatgattggaatgaggtgaacctggccgacgccgctggccggcatcgcgagctcattccggatggccaactgtgcagcgccgggcgggagaagtatcagggcctcgacctggcacgctccgactggacagccacttccttgtcctccggcgtctccttcacatacctctacaaggccaccgccccgcacttgggcttcttcgagttctacgtcaccaaggatggttacgagcccactgagccgctcaaatgggcagacttggaggactcgcccttcatcaacgtcaccgaccccacgcttgtcagcggctcctaccaaatccccggcaccacgccttccggcaagtccggccgccacctcatctacgtcatttggcagcgctccgacagccccgaggccttctactcctgctccgacgtcgacttcgacgtcgatgccctctctctccactccaccacc

SEQ ID NO: 17 - DNA, 738 bp, Platycerium superbum
atggagaagttatctgaggtggaggaaaagtggataatggagagttggcagtgggcgaaggtgctgatgcaggtgagggtgagggtgaggatgaggaggtcatgggtagctgtggctgttaccttggtggtgtgcgccggcagcctgctgggcgtagcgagcggtcatggcagcatggaggatcccatcagccgcgtctatgggtgctacctggagaatccggagaatcctacgtcggcagcgtgcatcgcggcggtggcggcaagtggcactcaagccttctacgactggaatgaggtgaatcagccctttgccgctggccaacaccgccagatcattcctgacggccagctctgcagcgccgggcgggacaagtataaaggcctcgacctggcacgcgccgactggcctgccacctccttatcttcgggcgtcgattacacttttctcttcaaggccaccgccccccaccggggctacttcgagttctacgtcacccgcgatagctacgaccccactgagcccctggcctgggccgacctggaggacacgcccttcatcaacgtcaccgacccgacccttgtgagcggctcctatcagatctccagcaccacgccttccggcaagaccggccgtcacctcatctacgtcatttggcagcgcaccgacagcactgaggccttctactcctgctccgatgtcgactttgacgagaccctccgccttcactccgccacc

SEQ ID NO: 18 - DNA, 714 bp, Davallia tyermannii
atgtggagcatgcatttgtgtggagtaaggaggatcttgagacaaggcaaaatcggtcatagtgtgagaatggggaggtcatggggagttgtggctattatggtgatgtacattggtggcctgctaagcatagcaagcggccatggcagcatggaggaccccatcagccgcgtctataggtgctacttggagaatccggagagtcccacatcggcagcttgccaagcggcagtggcagtgagtggggcccaagccttctacgattggaatgaggtgaacattgctgacgccaatggccggcaccgcgagctcatttccgatggccacctatgtagcgccaatcgaactaagtatgcaggcctcgacctggcatgccccgattggctaggcaccctcttgttctcgggcgtctcctacacattttcctacaaggccaccgcgccacacttgggcttctttgagttctacgtcacccgggatggttacgagcccaccgacccgctcaaatgggcagacttggaggactcgcccttcatcaacgtcaccaaccccacacttgataatggcgcctaccagatctccggcaccacgcctgccggtaagtcggggcgtcatctgatctacgtcatttggcagcgctctgatagcccagaggcattctattcgtgctccgacgtcgactttgtcgatgctctctctctccactctaccacc

SEQ ID NO: 19 - DNA, 723 bp, Tectaria milnei
atgcatcttggaatctgcaacattcgtgctgtagggaggatgagacaagccaatattggagatagtgtgaggatggggaggtcatggggagtggtggctgttatggtggtgtgcgcaagcggcctattgagcgtagtgaggggccatggaagcatggaggaccccatcagtcgtgtgtatgcatgcttcctagagaatccggagcgtcccatatcagcagcttgccaggcggcagtggcaatgggtgggacgcaagccttctatgattggaatgcggtaagcctgccctatgctgctgggcagcaccgtgaactcatcccggatggccaattgtgcagtgctgggcgggccaagtatcggggcctggacctgcctcgtgacgattggccaggcacctccaatatgacctccggcgtcgccttcacatacaggtacaaggccaccgccccacacttgggctccttccagttctatgtcactcgggatggctacgatcccaccgagccgctcaaatgggcagacttggaggactcgcctttcatgaacgccaccagcacgcttgccccggactcctacctaatgtccggcaccacccctagcggcaaggctggccaccacctcatctacgccatttggcagcgcagcgacagccctgaggccttctactcctgctccgatgtcaccttcgacgtcgctgctgtctctgatctccactccaccacc

SEQ ID NO: 20 - DNA, 720 bp, Cyrtomium falcatum; identical to SEQ ID NO: 15

SEQ ID NO: 21 - DNA, 720 bp, Polystichium tsus-simense
atgtgcaacaatatgcgtgcagtaattaggagtacgagacaattaggcaattatattggtcatagtgtgaggatggggaggtcatggtggggagttttggctgttatggtgttgtgcgccagcggcctgctgggcgtagcgagcggccatggcaccatgaatgaccccatcagccgcgtctacaactgcttcctggagaatccggagagccccacgtcggcagcttgcatagctgcggtggcgctgagtgggacccaagcgttctatgattggaatgaggtgaacctggccaacgccgctggccgacaccgcgagctcattccggatggccaactgtgcagcgccgggcgggacaagtataagggcctcgacctggcacgctccgactggacagccaccaacttgtcctccggcgtcgccttcacattcctctacagggtcaccgcccagcacaggggcttcttcgagttctacgtcaccgtggatgactacgaccccactgagctgctcaaatgggaagacttggaggaaacgccttttctcaacgtcactgaccccacggttgtaggcgtcaactatgaaatctccggcaccacgcctgccagcaagactggccgccacctcatctacgtcatttggcagcgctccgacagccccgaggccttctactcctgctccgacgtcgacttcgtcgatagcctctctctccactccaccacc

SEQ ID NO: 22 - DNA, 720 bp, Nephrolepis falcata
atgcatcatggaatctgcaacattcatgcaatagggaggaggagacaagccaatattggtcgtagtgtgaggatggggaggtcatggtggggagctgtggctattgtattggcggtgtgcgccagcggcctgctgagcgtagtgagcggccaaggaagcatggcgtaccccatcagtcgcgtctatggatgcttcctagagaatccgttgagtcccacgtcagcagcttgcaacgcggccgtggcattgagtgggacgcaagccttctatgattggaatgaggtgagcctggccaatgcctctggccagcaccgccaactcattccggatggtcagttgtgcagtgccgggcaggccaagtatcggggcctcgacctggctcgcgacgattggccaggcacctccttgacctccggtgtcgcctacacattctactactatgccaccaccctgcacttgggcttcttcgagttctatgtcactcgggatggctacgatgccacccagcccctcaaatgggcagatctggaggactcgcctttcctcaacgtcaccagcacgcttgccgcctcctccttccagtggtctagcatcactcccagtgacaagtctggccgccacctcatctacgtcatttggcagcgcaccgacagccctgaggccttctactcctgctccgacgtcgacttcgactatgccgtctctctccactccaccacc

SEQ ID NO: 23 - DNA, 717 bp, Nephrolepis exaltata
atgcatcttggaatctgcaacattcgtgcaatagggaggaggagacaagccaatattggtggtagtgtgaggatggggaggtcatggggagttgcggctattgtagtggcggtgtgcgccagcggcctgttgagcgtagtgagcggccatggaagcatgcaggaccccatcagtcgcgtctatgcatgctacctagagaatccggagcgtcccacgtcagcagcttgccaggcggcagtggcattgagtgggacgcaagccttctatgattggaatgaggtgaacctgcccaatgccgctggccggcaccgcgaactcattccggatggtcagttgtgcagtgctgggcgggccaagtatcagggcctcgaccaggctcgcaacgattggccacacaccgacttgatctccggcgtcgccttcacattcaactacagggccaccgccccacacttgggcatcttcgagttctatgtcactcgggatgggtacgatgccacccagcccctcaaatgggcagatctggaggactcgcctttcctcaccgccaccagcacgcttgccccctcctcctaccagtggcccggcaccactcccagtggcaagtctggccgccacctcatctacgtcatttggcagcgcaccgacagccccgaggccttctactcctgctccgacgtcgagttcgtcgatgccgtctctctccactccaccacc

SEQ ID NO: 24 - DNA, 717 bp, Nephrolepis exaltata
atgcatcttggaatcttcaacattctggcaatagggatgagtatgcaagccaatattggtggtagtgtgaggatggggaggtcatggggagttgcggctattgtagtggcggtgtgcgccagcggcctgttgagcgtagtgagcggccatggaagcatgcaggaccccatcagtcgcgtctatgcatgctacctagagaatccggagcgtcccacgtcagcagcttgccaggcggcagtggcattgagtgggacgcaagccttctatgattggaatgaggtgaacctgcccaatgccgctggccggcaccgcgaactcattccggatggtcagttgtgcagtgctgggcgggccaagtatcagggcctcgaccaggctcgcaacgattggccacacaccgacttgatctccggcgtcgccttcacattcaactacagggccaccgccccacacttgggcatcttcgagttctatgtcactcgggatgggtacgatgccacccagcccctcaaatgggcagatctggaggactcgcctttcctcaccgccaccagcacgcttgccccctcctcctaccagtggcccggcaccactcccagtggcaagtctggccgccacctcatctacgtcatttggcagcgcaccgacagccccgaggccttctactcctgctccgacgtcgagttcgtcgatgccgtctctctccactccaccacc

SEQ ID NO: 25 - DNA, 744 bp, Humata termanii
atgagtatatatatacacacaaatgttcgaatgtggagcatgcatttgtgtggagtaaggaggatcttgagacaaggcaaaatcggtcatagtgtgagaatggggaggtcatggggagttgtggctattatggtgatgtacattggtggcctgctaagcatagcaagcggccatggcagcatggaggaccccatcagccgcgtctataggtgctacttggagaatccggagagtcccacatcggcagcttgccaagcggcagtggcagtgagtggggcccaagccttctacgattggaatgaggtgaacattgctgacgccaatggccgacaccgggagctcatttctgatggccaactatgtagcgcaaatcggagtaagtatgcgggcctcgacctggcacgcgcagattggctaggcaccaccttgtcctcgggcgcctccttcacatttgcctacaaggccaccgcgccgcacttgggcttctttgagttctacgtcacccgggatggttacgagcccaccgacccgctcaaatgggcagacttggaggactcgcccttcatcaacgtcaccaaccccacacttgataatggcgcctaccagatctccggcaccacgcctgccggtaagtcggggcgtcatctgatctacgtcatttggcagcgctctgatagcccagaggcattctattcgtgctccgacgtcgactttgtcgatgctctctctctccactctaccacc

SEQ ID NO: 26 - DNA, 747 bp, Adiantum tenerum (Scutum Roseum)
atgactcaaggtgtttcgaatttgcatacgaatcatcttacggtccttaggtcacctagctttattggtcgtagtgtgagtgttagtatgggctggtgcaggtcatggggagttgtggctgtgatggtgttgtgcaccagcggcctcctgggcgtagcgagcgggcatggcagcatgaaggaccccatcagccgcgtctacaactgctacctggagaatccggagaggcccacgtcggcagcttgccaagcggcggtggcgctgagcgggacccaagcattctatgattggaatgaggtgaacctgcccaacgccgcgggtcggcaccgtgagctcattccggatggcgaactgtgcagcgccgggcgggaaaagtatcagggcctcgacctggcgcgcgccgactggacagccacgtccttgacctccggcctcgactcgttcacatggctctacaaggccaccgctccgcacttgggcttcttcgagttctacgttacccgggacggttacgacccgaccgaggcgctcacatgggcagacctggaggactcgccgttcataaacgtcaccaaccccgcgcttgtcagcggcgactaccaaatctccggcaccatacctgccggcaagagcggccgccacctcatctacgtcatttggcagcgctccgacagcccggaggccttctactcctgctccgacgtcgacttcgtcgatgatgccctgatctctctccgctccgccaca

SEQ ID NO: 27 - DNA, 723 bp, Polystichum setiferum (compacta)
atgtatatatgtgaaatgcatgttggaatgtgcagcaatatgcgtgcagtagttagacacggcaatcatagtgtgaggatggggaggtcatggggagttgcggctattatggtgttgtgcgccagcggcctgctgggtgtagcgagcggccatggcaccatgcatgaccccatcagtcgtgtctacaactgcttcctggagaatccagagagtcccacgtcggcagcttgcatagaggcggtggaggtgagtgggacccaaccattctatgattggaatgaggtgaacctggccaacgccgctggccggcaccgcgagctcattccggatggcaaactgtgcagcgccgggcgggacaagtataagggcctcgacctggcacgctccgactgggtagccaccaacttgtcctccggcgtcgccttcacattcctctacagggtcaccgccgagcacaggggcttcttcgagttctacgtcaccgtggatgattacgaccccactgagctgctcaaatgggaagacttggaggaaacgccgttcatgaatgtcaccgaccccacggttgtaggcgccaactacgaaatccccggcaccacgcctgccaacaagaccggccgccatctcatctatgtcatttggcagcgctccgacagccccgaggccttctactcctgctccgacgtcgtcttcgccgatgccgtgtctctccactccaccacc

SEQ ID NO: 28 - DNA, 723 bp, Polystichum setiferum (compacta)
atgtatatatgtgaaatgcatgttggaatgtgcagcaatatgcgtgcagtagttagacacggcaatcatagtgtgaggatggggaggtcatggggagttgcggctattatggtgttgtgcgccagcggcctgctgggtgtagcgagcggccatggcaccatgcatgaccccatcagtcgtgtctacaactgcttcctggagaatccagagagtcccacgtcggcagcttgcatagaggcggtggaggtgagtgggacccaaccattctatgattggaatgaggtgaacctgcctgacgtcaatggccggcaccgcgagctcattccagatggcaaactgtgcagcgccgggcgggagaagtataagggcctcgacctggcacgctccgactgggtagccaccaacttgtcctccggcgtcgccttcacattcctctacagggtcaccgccgagcacaggggcttcttcgagttctacgtcaccgtggatgattacgaccccactgagctgctcaaatgggaagacttggaggcaacgccgttcatgaatgtcaccgaccccacggttgtaggcgacaactacgaaatccccggcaccacgcctgccaacaagaccggccgccatctcatctatgtcatttggcagcgctccgacagccccgaggccttctactcctgctccgacgtcgtcttcgccgatgccgtgtctctccactccaccacc

SEQ ID NO: 29 - DNA, 729 bp, Lepisorus bicolor
atgtcctggggagttgtggctattatggtggccgtgtgtgccagcggcctgcttttggtaattattttttatagaagtgtgaggatgaggtcctggggagttgtggctattatggtggccgtgtgtgccagcggcctgctgggcgtcgcgagtggccatggcagcatgtcggaccccatcagtcgcgtctataggtgccgcctcgagaatccggagcgtcccacgtccgcagcctgcatcgcggcggtggcgcttagcggcaagcaagccttctacgattggaatgaggtgaatctgcccttcgccaatggccggcaccgcgagctcatccctgacggtaaactttgcagcgccgggcgggacaaatataaaggcctcgacctgccacgcgccgactggctggccacctccttgtcttctggctccgcctacacattcctctaccgggccaccgccccccacctgggctactttgagttctacgtcacgcgggatagctacgaccccactcagccgctcgcatggtcggacttggaggactcgccgttcatcaaggtcaccaacccgcccctcgtcagcggattttacgaatttcctggcaccacgccttccggcaaaaccggccgccacctcatctacgtcatttggcagcgcaccgacagcaccgaggctttctactcctgctccgacgtcgactttgacgaggccctctctctttcctccaccatc

SEQ ID NO: 30 - DNA, 750 bp, Pyrrosia lingua
atgagatcctgtataaaaagggcgggactggaaaggaggagcagcagcgaagatcctgagagacatctggtgctttttagatacagagtgtgtgagaggatgaggacgagggtatggggagttgtggcttttatggtggccgtgtgtgcctgcgacctgctgggcctagcgagtgggcatggctccatgggggaccccgtcagtcgcgtattgaattgctacctcgagaatccggagaggcccacgtcggcagcctgcatcgcggcggtggcgctgagtggcacccaagctttctacgactggaatgaggtgaacctggcctccgcctgtggccggcaccgcgagctcatttctgacggcgaactctgcagcgccgggcgcgacaagtataaaggcctcaacctggcacgcgccgactgggtggccacctccctgtcttcgggcgtcgattacacattcctctttaacgccaccgccgcccacctgggctacttcgagttctgggtcacccgtgatagctacgaccccactcagccgctcgcctgggcggacttggaggactcgccattcatcaacatcaccaaccccaccattgtcagcgatgcctaccaagtgcccgccaccacgccttccggcaagaccggccgccacctcatctacgtcatttggcagcgcactgacagcaccgaggccttctactcctgctccgacgtcgactttgacgaggccctccctctctcctccaccacc

SEQ ID NO: 31 - DNA, 735 bp, Blechnum appendiculatum
atgcaggacccccgactcacagtttatcttatctgcatgtatacactcactgatctgattaggatgaagaagtcatccggagttgtagtagtggtagtagcagctatattactgttgtgcctgctgggcgtggcaaacggccatggcagcatgcaggaccccatcagtcgcgtctacaactgcttcctagagaacccggagagtccgacatcggcagcttgccaagctgcggtagcagtggccgggacgcaaccattctacgattggaatgaggtgaacctggccaacgccaatggccggcaccgcgagctcatttcagatggcatgctgtgcagcgccaaccggtccaagtatcatggcctcgacctggcgcgcgccgactggacggccacctccttatcctctggcgtcgcctacacattcctgtaccgggtcaccgcccaccacaggggtttcttcgagttctacatcacccgtgacagctacgaccccacccagccgctcgcatgggcagacctggaggactcaccgttcatcaacattaccgaccccacgactgtgagtacgactctgggtgaagcctacgaaatctccggcaccacgcccgccagcaagagcggtcgccacctcatctatgtcatctggcagcgcagcgacagccccgaggcattctactcctgctccgacgtcgacttctctgccgatgccctgatctctctccgctccgcagtactc

SEQ ID NO: 32 - DNA, 717 bp, Polystichum munitum
atgcatcttggaatgtgcagcaatatgcgtgcagtaattacacaaggcaattatattggtcatagtgtgaggatggggaggtcatggggagttgtggctattatggtgttgtgcgctagcggcctgctgggcgtagcgagcggccatggcaccatgaacaaccccatcagccgcgtctacaactgccgcctggagaatccggagcgtcccacgtcagcagcttgcatagcggcggtggcgctgagtgggacccaagcgttctatgattggaatgaggtgaacctgcccgacgtcaatggccggcaccgcgagctcattccggatggcaaactgtgcagcgccgggcgggacaagtataagggcctcgacctggcacgctccgactgggtagccaccaacttgtcctccggcgtcgccttcacattcctctacagggtcaccgcccagcacaggggcttcttcgagttctacgtcaccgtggatgattacgaccccactgagctgctcaaatgggaagacttggaggaaacgccattcatgaacgtcaccgaccccacggttgtaggcgtcaactacgaaatcccaggcaccacgcctgcaaacaagaccggccgccatctcatctatgtcatttggcagcgctccgacagccccgaggccttctactcctgctccgacgtagacttcgtcgatgccgtgtctctccactccaccacc

SEQ ID NO: 33 - DNA, 696 bp, Stenochiaena tenuifolia
atgaggcgacacaatactggttataatagtgagcgagcactgtgcatggggatggggaggtcaaactcatctaaagttgtagctatcgtggtgttgtgcagtggcctgctgagcctagtgagcggccatggcagtatgcagaaccccatcagtcgcgtcctcaactgctacctggagaatccggagcgtcccacgtcggcagcttgccaagcggcggtggcgatgagtgggacccaagccttctatgattggaatgaggtgaacctgcccaacgccgctggccggcaccgccaactcattcccgatggccaactgtgcagcgccgggcggcagaagtatcggggcctcgacttggctcgcgacgactgggaagccaccaccttgtcctccgggaccgccttcacatacaactacagggccaccgccccgcacctgggcttcttcgagttctacgtcactcgggatggctacgagcccactgagcctctcaaatggtccgacttgcaggactcgcccttcatcaacgtcaccaccacgctttctagcgactcctaccaaatcaccggcaccacgcctgctggcaagtccggccgccacctcatctacgtcatttggcagcgctccgacagccccgaggccttctactcctgctccgacgtcgagttcgacgttgccctctctctccattccgccacc

SEQ ID NO: 34 - DNA, 693 bp, Asplenium bulbiferum (G.Forst.)
atgagaatggggagatcgacatcttgcatgggagcaaatatggctttcatgctgctgctgctgttgttttgggctagctgctgctgcctgctgggcaaagtgagcgggcatggcagcatggaggatcccatcagccgtgtctacgcctgcttcttggagaatccggagaggccgacgtcggcagcatgccaagcggcggtggcgttgagtgggacgcaagcgttctatgattggaacgaggtcaaccagcccaacgctgccggccggcaccgcgagataatcccggacggccagctctgcagcggcgggcgggagaagtatcagggcctcgacttggcacgtgacgactggacggccacctccttgtccccaaacgtctccttcacgttcctctacaaggcgacagcgcctcaccgcggtttcttcgagttctacgtcacccgggatggttacgaccctaccgaggccctcacatgggccgacttggaggaaccgccattcatcaacgtcaccgaccccacggttgcctccggcgcctaccagatccccggcaccacaccggccggcaagactggccgccatctcatctacgtcatatggcagcgctctgatagccccgaggccttctactcttgctccgacgtcgacttcgagagtgccgataccgtcaatatctctctccgctctaccacc

SEQ ID NO: 35 - DNA, 699 bp, Athyrium filix-femina
atgaatattgcaggtcatactagtgtgagggtgaggatggggaggtcatggggagttgtggctattcttatggtgttgtgcggctgcctgctgggcgtagcgagcgggcatggcagcatggaggaccccatcagtcgcgtctacaactgctacctcgagaatccggagagtcccacgtcggcagcttgccaagcggcggtggcgctgggtgggccccaaccgttctatgattggaatgaggtgaaccagcccaacgccgatggccactcccgcgagatcattccggatggccaactgtgcagcggcgggcgggagaagtataagggcctcgacctggcacgctccgactggacagccacctccttgtcctccggcgtcgccttcacattcctcttcaaggccactgccccgcacgcgggcttcttcgagttctacgtcacccaggatggttacgaccccactgagccgctcaaatgggcagacttggaggactcgcccttcatcaacgtcaccgaccccacgcttctcagcggctcctaccaaatccccggcaccacgcctgccggcaagtccggccgccacctcatctacgtcatttggcagcgctccgacagccccgaggccttctactcctgctccgacgtcgacttcgtcgatgccctctctagtgatctccactccaccatggcaccaatagct

SEQ ID NO: 36 - DNA, 693 bp, Adiantum capillus-veneris
atggggatgaagatgtcatgggaagttgcactagcagaaatagtagctttgtgcctactgggcatggcaagcagccatggcaccatgcaggaccccataagtcgtgtctacaactgctttctggagaacccggagaggccaacgtcggcagcttgtcaagctgcagtagcgttgggtggcacacaaccactctatgattggaatgaggtgaacatccatgatgccgctggcaaccaccgcgatctcatccccgatggcaagctctgcagcgccggccgccaaaagtttcagggcctcgacttggcgcgcgcggattggatagcaacctccctatcctctggcgtcgacgtcgactacacattcctctaccgcgccaccgccccgcacttgggcttctttgaattttacatcacccgtgacacctacgaccccacccagccgctcgcatggggtgacctggaagactcgcccttcatcaacattaccaatccctccatcgtcagtacgactttgggtcccgcctactcgatccccagcactacaccattcagcaaaagtggtcgccacctcatctacgtcatctggcagcgcaccgacagcctcgaggcgttctactcctgctccgacgtcgacttctcgacatcttccatcgaggatgatgtcatcgtctctctccgttctgcagctctactc

SEQ ID NO: 37 - DNA, 699 bp, Coniogramme emeiensis (Golden Zebra)
atgtatacactcactgatctgattaggatgaagaagtcatccggagttgtagtagtggtagtagcagctatattactgttgtgcctgctgggcgtggcaaacggccatggcagcatgcaggaccccatcagtcgcgtctacaactgcttcctagagaacccggagagtccgacatcggcagcttgccaagctgcggtagcagtggccgggacgcaaccattctacgattggaatgaggtgaacctggccaacgccaatggccggcaccgcgagctcatttcagatggcatgctgtgcagcgccaaccggtccaagtatcatggcctcgacctggcgcgcgccgactggacggccacctccttatcctctggcgtcgcctacacattcctgtaccgggtcaccgcccaccacaggggtttcttcgagttctacatcacccgtgacagctacgaccccacccagccgctcgcatgggcagacctggaggactcaccgttcatcaacattaccgaccccacgactgtgagtacgactctgggtgaagcctacgaaatctccggcaccacgcccgccagcaagagcggtcgccacctcatctacgtcatttggcagcgcagcgacagccccgaggcattctactcctgctccgacgtcgacttctctgccgatgccctgatctctctccgctccgcagtactc

SEQ ID NO: 38 - DNA, 693 bp, Asplenium nidus var plicatum
atgagaatggggagatccatatcacgcatggcagctaggatggctattatgctggtgttgtgctgggctataagctgctgcctgctgggcacagtgagcgggcatggcagctctgaggatcccatgagccgtgtctatgggtgctacttgcagaatccggagaggcccgcatcggcagcctgccgagcggcagtggcgatgagtgggacgcaagcgttctatgattggaacgaggtcaaccagccccatgctgccggtcggcaccgcgagatcattccggatggccagctctgcggcggcgggcgggcgaagtatcggggcctcaacttggcacgtgccgactggtggtccacccccttgtactccaacacccccttcatgttcctctatagggctaccgcccctcacaggggtttcttcgagttctatgtcacccgggatggttacgatcccactgaacccctcaaatggtcggacttggagtacccaccattcatcaacgtcaccgaccccacgcttgccttcggcgcctacaagatccccggcttcacaccgtatggcaagactggccgccatctcatctacatcatatggcaacgctctgatagcccagaagccttctactcttgctccgacgtggacttcgtggacttcaagagcgatgaaaccgtgatccctctccactctaccacc

SEQ ID NO: 39 - DNA, 693 bp, Polystichum polyblepharum
atgcttgcagtaattagacaaggcaattatattggtcatagtgtgaggatggggaggtcatggggagttgtggctattatggtgctgtgcgctagcggcctgctggacgtagcgagcggccatggcagcatgaacgaccccatcagccgtgtctacaactgccgcctggagaatccggagagtcccacgtcagatgcttgcatagcggcggtggcgctgagtgggacccaagcgttctatgattggaatgaggtgaacctgcccaacgccgctggcaggcaccgagagctcattccggatggcaaactgtgcagcgccgggcgggacaagtataagggcctcgacctcgcacgctccgactgggtagccaccaacttgtcctccggcgtcgccttcacattcctctacagggtcaccgcccagcacaggggcttcttcgagttctacgtcaccgtggatgattacgaccccactgagctgctcaaatgggaagacttggaggaaacaccgttcatgaatgtcaccgaccccacggttgtaggcgtcaactacgaaatggccggcaccacgcctgccaacaagaccggccgccatctcatctatgtcatttggcagcgctccgacagccccgaggccttctactcctgctccgacgtcgacttcgtcgatgccgtgtctctccactccagcacc

SEQ ID NO: 40 - DNA, 699 bp, Adiantum venustum
atggggagacgtcgtgcagtaaggaaaggtcataatagtgtgaggaggatatccatggggaggtcatggggagacgttgtggctattatggtgttgtgcgccagcggcctgctgggcgtagcgagcggccatggcagcatgcaggaccccatcagtcgcgtctacaactgctacctggagggtccggagagtcccacgtcggcagcttgcatagcggcggtggcgctgagtgggacccaagcattctatgactggaatgaggtgaaccagcccaacgccgctggccggcaccgcgagatcatcccggatggccaactctgcagcggcgggcgggacaagtatagcggcctcgaccttgcgcgctccgactggacagccacctccttgtcctccaacgtctcctacacatacctcttcaaggccaccgccccgcacaagggcttcttcgagttttacgtcacccgggacagctacgagcccactgaggcgctcaaatgggcagacttggaggactcacccttcattaacatcaccgaccccacgcttgacagcggcgcctaccaaatccccggcaccacgcctgccggcaagtctgggcgccacctcatctacgtcatttggcagcgctccgacagcggcgaggccttctacgcctgctgcgacgtcgacttcgatgtcgatgtcctccactccaccaca

SEQ ID NO: 41 - DNA, 699 bp, Actiniopteris australis
atgaggcaaggcagtagtattgctgatatgagtgtgagaatggggggagttaacgctgttgctatcatattgctgttgtgctgcgctagcagcggcttgctgggcatagcccgcgggcatggcagcatgcaagatcccatcagccgtgtctacgcctgctacttggagaatccggagcgtcccacatcggcagcttgccaagcggcagtggccttgagtgggacgcaagccttctatgactggaacgaggtgaaccagccgtttgctgctggccgccaccgcgagatcattcccgacggccagctttgcagcggtgggcggaccaagtatgcgggcctcgacctggcacgcgacgactggacagccacctccttgtccgccggcatctcctacacattcctctacagaggcaccgccccgcaccttggcttcttcgagttctacgtcacccgggatggttacgatcccactgagcccctcaaatgggcagacttggaggacccgcctttcatcaacatcaccaaccccactcttgtcagcggcgtttaccagatccccgggaccacacctgccggaaagactggccgccatctcatctacgttatctggcagcgcaccgacagccccgaggcgttctactcctgctccgacgtcgtcttcagcgacgatgccgccctctatctccgctctaccactgag

SEQ ID NO: 42 - DNA, 693 bp, Marsilea crenata
atgaggaggagcgggatgagcagcagcgtgctagccgctgtcgccgccggagttcttctagtggcggcactaggcagccacgtggcgtacgggcacggcagcatgaaggaaccaatcagccgcgcttacaactgctacctcgaaattgctgacaatgccacgtcagacgcgtgcggggcggcggcagcgctttgcatccctgaagccttcaacgactggaacgctgtacttatccctgacgtcgccggccgccaccgccagctcatcccggacggacagctgtgcagcgccggaagagcgaagtacgccggcctgaatctcgcaagtgtggactgggaggccgccaccttggctgccggcgtgaactacacgtttctgtacaaggccgtagtggtccacaaaggctacttcgagttctacgtcaccaaggacggctacgacgccacgcaagcgctcacatggtccgacttggaagacgcccctttcgtcaacgtcaccgatcccatagtcaattccgacagtgacttcgaaattcccggcaccattccctccgggaagtccggccgccacgtgatctacgtcatttggcagcgcaccgacagccccgaagctttctactcctgctcggacgtcgacttcgacgacaccatctccgacgacaccatctccgacaccgtcctacatgccagctca

SEQ ID NO: 43 - DNA, 687 bp, Asplenium prolongatum x Asplenium antiquum (Kurata)
atgagaatggggaggtcggcatcttgcatcagagctaatatggctatcatgctggtgttgttttgggctagctgctgctgcctgctgggcatagtgagcgggcatggcagcatggaggatcccatcagtcgtgtctacgcctgctacttggagaatccggagcggcccacatctgcagcttgcatagcggcggtggcgttgagtgggacgcaagcgttctacgattggaacgaggttaaccagcccaacgccgccggtcggcaccgcgagatcattccggatggccagctttgcagcggtgggcgggagaagtatcagggcctcgacctggcacgtgccgactggacggccacctccctgacctccggtatcaccttcactttcctctacaaggcaacagcccctcaccgtggtttctttgagttctacgtcacccgcgatacttatgatcccaccgagcccctcacatgggcggacttggaggacacgccattcatcaacgccaccgaccccacgcttgcttccggctcctaccagatccccggcaccacaccagccggcaagactggccgccatctcatctacgtcatatggcagcgctctgatagccccgaagccttctactcttgctctgacgtggactttgagagcagcgataccgtgatctctctccgctctgccaccacc

SEQ ID NO: 44 - DNA, 687 bp, Adiantum raddianum (Fritz Luthi)
atggggatgaagatgtcatgggaagttgcactagcagaaatagtagctttgtgcctactgggcatggcaagcagccatggcaccatgcaggaccccataagtcgtgtctacaactgctttctggagaacccggagaggccaacgtcggcagcttgtcaagctgcagtagcgttgggtggcacacaaccactctatgattggaatgaggtgaacatccatgatgccgctggcaaccaccgcgatctcatccccgatggcaagctctgcagcgccggccgccaaaagtttcagggcctcgacttggcgcgcgcggattggatagcaacctccctatcctctggcgtcgactacacattcctctaccgcgccaccgccccgcacttgggcttctttgaattttacatcacccgtgacacctacgaccccacccagccgctcgcatggggtgacctggaagactcgcccttcatcaacattaccaatccctccatcgtcagtacgactttgggtcccgcctactcgatccccagcactacaccattcagcaaaagtggtcgccacctcatctacgtcatctggcagcgcaccgacagcctcgaggcgttctactcctgctccgacgtcgacttctcgacatcttccatcgaggatgatgtcatcgtctctctccgttctgcagctctactc

SEQ ID NO: 45 - DNA, 681 bp, Asplenium australasicum
atgagaatggggagatccacatcacgcatggcagctaggatggctattacgctgctgttgtgctgggctagctgctgcctgctgggcacagtgagcgggcatggcagcatgctggatcccatcagtcgcatctacgcctgcttcttggagaatccggagaggcccacatcggcagcctgccaggcggcagtggcgttgggtgggacgcaaccgctctatgattggaacgaggtcaaccagcccaatgctgccggtcggcaccgcgagatcattccggatggccagctttgcggcggcgggcgggagaagtatcagggcctcaacttggcacgtgccgactggccggcaacctccttgtcctccaacaccgccttcacgttcctctacattgctacagcccctcaccgcggtttcttcgagttctacgtcacccgggatggttacgatcccactgagctccttaaatgggcggacttggagtacccacccttcctcaacgtcaccgaccccacgcttgcctccggcaactaccagatccctggcaccacaccagccggcaagaccggccgccatctcatttacgtcatatggcagcgctccgatagccccgaagccttctactcctgctccgacatcgacttcgagagcgatgaaaccgtgatctctctccactctaccacc

SEQ ID NO: 46 - DNA, 681 bp, Asplenium australasicum
atgagaatggggagatccacatcacgcatggcagctaggatggctattacgctgctgttgtgctgggctagctgctgcctgctgggcacagtgagcgggcatggcagcatgctggatcccatcagtcgcatctacgcctgcttcttggagaatccggagaggcccacatcggcagcctgccaggcggcagtggcgttgggtgggacgcaaccgctctatgattggaacgaggtcaaccagcccaacgctgccggccgccaccgcgagatcattcccgatggccaactttgcagcggcgggcgggagaagtataagggcttcgacttgcctcgtgccgactggccggcaaccaccttggtctccaacatcagcttcacatacctctacaaggcaacagctcctcaccgtggtttcttcgagttctacgtcacccgggatggttacgatcccactgagctccttaaatgggcggacttggagtacccacccttcctcaacgtcaccgaccccacgcttgcctccggcaactaccagatccctggcaccacaccagccggcaagaccggccgccatctcatttacgtcatatggcagcgctccgatagccccgaagccttctactcctgctccgacatcgacttcgagagcgatgaaaccgtgatctctctccactctatcacc

SEQ ID NO: 47 - DNA, 687 bp, Adiantum raddianum (Gracillimum); identical to SEQ ID NO: 44

SEQ ID NO: 48 - DNA, 684 bp, Thelypteris palustris
atgaggcaaggcaattatataggtcatagtgtgaggatggggaggtcatggggagttgtgggtattatggtgttgtgcctgctgggcgtagcgagcggccatggcaccatgcaggaccccatcagtcgcgtctacaactgccgcctggagaatccggagcgtcccacgtcggcagcttgcatagcggccgtggcgctgagtgggacccaagcgttctatgattggaatgaggtgaacttggccaacgccgctggccggcaccgcgagctcattccggatggccaactgtgcagcgccgggcgggtcaagtaccagggcctcgacctggcacgctccgactggacagccacctccttgtcctccggcgtctccttcacattcctctacagggtcaccgcccagcacttgggcttcttcgagttctacgtcacccaggatggttacgaccccactgagccgctcaaatgggcagacttggaggactcgccgttcatcaacgtcaccaaccccacggttgtcagcacctccctaggccccgcctaccaaatcgctggcaccacgcctgccggcaagtctggccgccacctcatctacgtcatttggcagcgctccgacagccccgaggccttctactcctgctccgacgtcgacttcgtcgatgccctctctctccactccactgcc

SEQ ID NO: 49 - DNA, 687 bp, Adiantum raddianum (Variegatum); identical to SEQ ID NO: 44

SEQ ID NO: 50 - DNA, 690 bp, Asplenium dimorphum X Asplenium difforme
atgagaatggggagatcgacatcttgcatgggagctaatatggctatcgtcctgctgctgctgttgttttgggctagctgctgctgcctgctgggcaaagtgagcgggcatggcagcatggaggatcccatcagtcgtgtctacgcctgcttcctggagaatccggagaggccgacgtcggcagcctgccaagcggcggtggcgttgagtgggacgcaagcgttctatgattggaacgaggtcaacctgcccaacgctgccggccggcaccgcgaaatcatcccggacggccagctttgcagcggcgggcgggagaagtataaaggcctcgacttggcacgtgccgactggacggccacctccttgtccccaaacgtctccttcacgttcctctacaaggggacagcgcctcaccgcggtttcttcgagttctacgtcacccgggatggttacgaccctaccgaggccctcacatgggccgacttggaggaaccgccattcatcaacgtcaccgaccccacgcttgcctccggcgcctaccagatccccggcaccacaccagccggcaagacgggccgccatctcatctacgtcatatggcagcgctctgacagccccgaagccttctactcttgctccgacgtcgacttcgagagtgacgataccgtggtctctctccgctctaccacc

SEQ ID NO: 51 - DNA, 687 bp, Matteuccia struthiopteris
atgcttgcagtaaggaaaggcaatattggtgatagcgtgaggatggggaggtcatggggtgttgtagctattatggtgttgtgcgccagcagcctgctgggcgtagtgagcggccatggcagcatggcggaccccatcagtcgtgtctatgggtgccgtctggagggtccggagagccccacatcggcagcttgccaagcggcggtggcgctgagtgggacccaagcgttctatgattggaatgaggtgaaccagcccttcgccgctggccggcaccgcgagctcattccggatggccaactgtgcagcggcgggcgggtcaagtatcagggcctcgacctggcacgctccgactggccagccaccaacttgtcctccggcgtctccttcacattcctctacgaggtcaccgccacgcacttgggctactttgagttctacgtcacccgggatggttaccagccgactgagccgctcaaatgggcagacttggaggactcgccgttcctcaccgccaccacaacgcatgagagcagctcctacataatccctggcaccacgccttccgccaagtccggccgccacctcatctacctcatttggcagcggaccgacagccccgaggccttctactcctgctccgacgtcgacttcgtcgatgccctctctagtctccactccaccaac

SEQ ID NO: 52 - DNA, 684 bp, Athyrium filix-femina (angustum)
atgatgaatattgcaggtcatactagtgtgaggatggggaggtcatggggagttgtggctattcttatggtgttgtgcggctgcctgctgggcgtagcgagcgggcatggcagcatggaggaccccatcagtcgcgtctacaactgctacctggagaatccggagagtcccacgtcggcagcttgccaagcggcggtggcgctgggtggcacccaaccgttgtatgattggaatgaggtgaaccagcccaacgccgctggccagtcccgcgaaatcattccggatggccaactgtgcagcggcgggcgggagaagtatcagggcctcgacctggcacgctccgactggacagccacctccttgtcctccggcgtcgccttcacattcctcttcaaggccaccgccccgcacttgggcttcttcgagttctacgtcacccaggatggttacgaccccactgagccgctcaaatgggcagacttggaggactcgcccttcatcaacgtcaccgaccccacgcttctcagcggctcctaccaaatccccggcaccacgcctgccggcaagtccggccgccacctaatctacgtcatttggcagcgctccgacagccccgaggccttctactcctgctccgacgtcgacttcgtcgatgccctctctagtgatctccactccaccacc

SEQ ID NO: 53 - DNA, 687 bp, Adiantum monocolor; identical to SEQ ID NO: 44

SEQ ID NO: 54 - DNA, 684 bp, Adiantum pubescens (Bronze)
atgaagaagtcttggggagttacagctgtagtgggagtaatagctttgtgcctgctggacgtggcaagcggccatggcagcatgcaggaccccatcagtcgtgtctacaactgctttctagaaaacccggagcgcccaacgtcggcagcttgcatagctgcggtggcaatgagtggcacacaaccattctacgattggaatgaggtgaacttggccgacgccaatggccggcaccgcgagctcatccccgatggcaagctgtgcagcgccggcagggataagtatcagggcctcgaccaggcgcgcgacgactgggtagcaacctccttatcctctggcgtcgcctacacattcctttaccgggtcactgccccgcacttgggcttctttgaattttacgtcacccgtgacacctacgaccccactcaggcgctcgcatgggatgacctggaagactcgcccttcatcaacattaccaacccctccgttgtcagtacgacgttgggtaacgcctactcaattcccggcaccacgccatccggcaagactggtcgccacctcatctacgtcatctggcagcgcagcgacagtcgcgaggcgttctactcctgctccgacgtcgacttcccggcatcgacagtcgaggatgacgtcatcatctctctccgctccgcagctctagtc

SEQ ID NO: 55 - DNA, 681 bp, Blechnum niponicum
atgagcgcagtaaggaatattggtcatagtgtgaggatgggaaggtcatggggagttgtggctattatggtgttgtgcgccagcggcctgctgggcgtagcgagcggccatggcagcatggacgaccccatcagtcgtgtctacaactgctacctggagaatccggagcgtcccacgtcggcagcttgccaagccgcggtggcgctgagtgggacccaagcgttctatgattggaatgaggtgaaccagcccttcgccgctggccggcaccgcgagatcattccggatggccaactgtgcagcggcgggcgggagaagtatcagggcctggacctggcacgctccgactggacagccacctccttgtcctccggcgtctccttcacatacctgtacaaggccaccgccccgcacttgggcttcttcgagttctacgtcaccgtggatggttaccagcccactgagccgctcaaatggtcagacttggaggacccgccgttcatcaacgtcaccaaccccacgcttgtcagcggctcctaccaaatccccggcaccacgcctgccggcaagaccggccgccacctcatctacgtcatttggcagcgctccgacagccccgaggccttctactcctgctccgacgtcgacttcgccgatgccctctctctccactccaccacc

SEQ ID NO: 56 - DNA, 672 bp, Platycerium wandae
atgtatggtggtcagcatactgggaggatggggaagccgtggagagtggtggtggccattgtggtggtgtgcgccagcggcctgctgggcgtagcgagcggccatggcagcatgggtgaacccatcagtcgcgtctataattgctacctggagaatccggagagacccacgtcggcagcgtgcatcgcggcggtggcgcttagtggcacccaagccttctacgactggaatgaggtgaacctgcccttcgccgctggccggcaccgcgagctcattcctgacggccagctctgcagcgccgggcgggacaagtataaaggcctggacctggcacgcgccgactgggttgccacctccctgtcttcgggcgtcagctacaccttcctctacagggccaccgccccccaccagggctactttgagttctacgtcaccaaggatagctacgaccccactgagccgctggcctgggcggacctggaggacacgcccttcattaacatcaccgatccgacccttgtcagcggctcttaccagatccccagcaccacgccttccgacaagaccggccgccacctcatctacgtcatttggcagcgcaccgacagccctgaggccttctactcctgctccgatatcgactttgacgacaccctccccctacactccacc

SEQ ID NO: 57 - DNA, 675 bp, Nephrolepis cordifolia (Duffii)
atgaaacaagccaatattggtcatagtgtaaggatggggaggtcatggcgagttgtggctattatggtggtgtgcgccagcggcctattgagtgtagtgaggggccatggaagcatggaagacccccttagtcgcgtctatgggtgcttcctagagaatccagagagtcccacgtcagcagcttgccaagcggcagtggcaatgagtgggaccctagctttctatgattggtttgatgtgagcttgcccaatgcttctggccggcaccgcgaactcattccggatggccaattgtgtggtgctgggctgaccaagtatcagggcctcaacctggctcgcgatgattggacagccacctccttgacctccggcgtctccttcacatacctctacaaggccgccgcccgacacttgggcttctttgagttctatgtcactcgggatggttacgatcccaccgagccgctcaaatgggcagacttggaggacttgcctttcatgaacgtcaccagcacgcttgacgaggagtcctaccaaatccctggcaccactcctagtggcaaggctggccgccacctcatctacgtcatttggcagcgcagcgacagccctgaggccttctactcctgctccgatgtcgacttcgtcgatgctgtctctctccactccaccacc

SEQ ID NO: 58 - DNA, 672 bp, Adiantum raddianum (Fragrans)
atggggatgaagatgtcatgggaagttgcactagcagaaatagtagctttgtgcctactgggcatggcaagcagccatggcaccatgcaggaccccataagtcgtgtctacaactgctttctggagaacccggagaggccaacgtcggcagcttgtcaagctgcagtagcgttgggtggcacacaaccactctatgattggaatgaggtgaacatccatgatgccgctggcaaccaccgcgatctcatccccgatggcaagctctgcagcgccggccgccaaaagtttcagggcctcgacttggcgcgcgcggattggatagcaacctccctatcctctggcgtcgactacacattcctctaccgcgccaccgccccgcacttgggcttctttgaattttacatcacccgtgacacctacgaccccacccagccgctcgcatggggtgacctggaagactcgcccttcatcaacattaccaatccctccatcgtcagtacgactttgggtcccgcctactcgatccccagcactacaccattcagcaaaagtggtcgccacctcatctacgtcatatggcagcgcagcgacagccccgaagctttctatgcctgctccgacatcgacttctccacttcttccgacatgatttctctccgctccgcagttctc

SEQ ID NO: 59 - DNA, 675 bp, Platycerium bifurcatum (Netherlands)
atgtatggtggtcagcatactgcgagcatggggaagccgtggagagtggtggtggccattgtggtggtgtgcgccagcggcctgctgggcgtagcgagcggccatggcagcatgggggatcccatcagtcgcgtctataattgctacctggagaatccggagaggcccacatcggcagcgtgcatcgcggcggtggcgcttagtggcacccaagccttctacgactggaatgaggtgaacctgcccttcgccgctggccggcaccgcgagctcattcctgacggccagctctgcagcgccgggcgggacaagtataaaggcctggacctggcacgcgccgactgggttgccacctccttgtcttcgggcgtcagctacaccttcctctacagggttaccgccccccaccggggctactttgagttctacgtcaccaaggatagctacgaccccactgagccgctggcctgggcggacctggaggacacgcccttcattaacatcaccgacccgaccattgtcagcggctcttaccagatctccagcaccacgccttccgacaagaccggccgccacctcatctacgtcatttggcagcgcaccgacagccctgaggccttctactcctgctccgatgtcgactttgacgacaccctccccctccactcctccacc

SEQ ID NO: 60 - DNA, 663 bp, Pyrrosia polydactyla
atgaggatggggatgaggatgaggttatggggagttgtggcttttatggtggccgtgtgtgccggcgagctgctggaccaagcgagtgggcatggctccatgggggaccccgtcagtcgcgtcttgaattgctacctcgagaatccggagaacccctcgtcggctgcctgcatcgctgcggtggcggcgagtggcacccaagccttctacgactggaatgaggtgaatctggccttcgccgctggccagcaccgcacgctcattcctgatggcgaactctgcagcgccggtcgggagaagtataaaggcctcaatctggcacgcgccgactgggtagccacttcattgtcttcaggcgccaactacacattcctctacagggccaccgccccccacctgggctacttcgagttctacgtcacgcaagatagctacgaccccactgagccgctcgcatgggcggacttggaggactcgccgttcatcaatgtcaccaacccggccctcgtcagcggctcctaccgaattgctggcaccacgccttccggcaaaaccggccgccacctcatctacgtcatttggcagcgcaccgacagccccgaggccttctactcctgctccgacgtcgactttgacgaggccgtctctctttcttccaccacc

SEQ ID NO: 61 - DNA, 666 bp, Blechnum brasiliense
atgaagaagccatggggagttgtagtagtagtagctatattactgttgtgcctgctgggcgtggcaagcggccatggcagcatgcaggaccccatcagtcgagtctacaactgctacctagagaacccagagaggccgacatcggcagcttgccaagctgcggtggcgatgagcgggacgcaagcattctacgattggaatgaggtgaacctggccaacgcttctggccggcaccgcgagctcattcctgatggcaagctgtgcagtgccggccgggacaagtatcggggcctcgacctggcgcgcgccgactggacggccacctccttatcctctggcgtcgcctacacattcctccaccgggtcaccgcccggcacttgggattcttcgagttctacatcacccgtgacagctacgaccccaccgagctgctcacatgggcagacctggaggactcgccgttcatcaacattaccaaccccacgactgtgagtacgtctctgggtaacgcctaccagatccccggcaccacgcccgccggcaagagcggtcgtcacctcatctacgtcatctggcagcgcagcgacagccctgaggcattctactcctgctgcgacgtcgacttctcttctgataccctgatctctctccgctctgcagcactc

SEQ ID NO: 62 - DNA, 666 bp, Blechnum sp. (Silver Lady)
atgaagaagccatggggagttgtagtagtagtagctatattactgttgtgcctgctgggcgtggcaagcggccatggcagcatgcaggaccccatcagtcgagtctacaactgctacctagagaacccagagaggccgacatcggcagcttgccaagctgcggtggcgatgagcgggacgcaagcattctacgattggaatgaggtgaacctggccaacgcttctggccggcaccgcgagctcattcctgatggcaagctgtgcagtgccggccgggacaagtatcggggcctcgacctggcgcgcgccgactggacggccacctccttatcctctggcgtcgcctacacattcctccaccgggtcaccgcccggcacttgggattcttcgagttctacatcacccgtgacagttacgaccccaccgagcccctcacatgggcagacctggaggattcgccgttcctcaacattaccgaccccacgactgtgggtacgcctctgggtgatgcctacgaaatccccggcaccacgcccgacggcaagagcggtcgccacctcatctatgtcatctggcagcgcagcgacagccctgaggcattctactcctgctgcgacgtcgacttctcttctgataccctgatctctctccgctctgcagcactc

SEQ ID NO: 63 - DNA, 669 bp, Pteris cretica (Mayi)
atggggtcgaggtcagtgggcggcggaggagctggggctatttattgtatgctgctaatatgctgcgttagcagcgggctgctgggcatagcgagcggccatggcaccatgctggacccctttagtcgtgtgtacgcctgccgcttcttcgagaatccggagcgtcccacatcgccagcatgccaagcagcagtggcggcgagtggaacgcaagcgttctatgactggaacgaggtgaaccagcccttcgccgctggccggcaccgcgagatcattccggacggccaactttgcagcggtgggcgggacaagtataagggcctcgacctggcacgcaacgactggccagccacctccttgtcctccaacatccccttcacatacctgtacattgccagcgctccgcaccgcggcttcttcgagttctacgtcacccaggatggttacgatcccactcagcccctcaaatgggcagatttggagtacccgccattcatcaacatcaccgaccccacgctgctcagcggctcctaccaaatccccggcaccacgccggccggcaagtctggccgccatctcatctacgtcatttggcagcgctccgacagccccgaggccttctactcctgctccgacgtcgacttcgtcgactctctccacgcctccgtc

SEQ ID NO: 64 - DNA, 663 bp, Cystopteris fragilis
atggggagagttaaccttctggctattctggtgttgtgcgccagctgctgcgccggcctgctgggcgtagccagcggccatggcaccatggaggaccccatcagtcgcgtctacaactgcttcctggagaacccggagcgtcccacgtcggcagcttgccaagcggcggttgcgctgagtggcacccaagcgttctatgactggaatgaggtgaacctggcggacgccgctggccggcatcgcgagctcattccggatggccaactgtgcagcgccgggcgggagaagtatcggggcctggacctggcacgctccgactgggtagccacctccttgtcctccggcgtctccaccacattcctctacaaggccacggctccgcacttgggcttcttcgagttctacgtcacccgggatggatacgaccccaccgaggcgctcaaatggtcagacttggaggactcgccgttcctcaacgtcaccgaccccacccttctcagcagcccctacgtctaccaaatccctggcaccacgcctgccggcaagtccggccgccacctgatctacgtcatttggcagcgctccgacagccctgaggccttctactcctgctccgacgtcgccttcgacgatgcccagcttgtctctctccactccaccacc

SEQ ID NO: 65 - DNA, 660 bp, Dryopteris filix-mas
atggggaggtcatggggagtggtgcaggctataattatggtgttgtgcggcagcggcctgctgggcgtagcgagcggccatggcagcatggaggaccccatcagtcgcgtctacaactgctacctggagaatcccgagagtcccacgtcggcagcttgccaagcggcggtggcgctgagtggggcccaagcgttctatgattggaatgaggtgaacctggccgacgccgctggccggcatcgcgagctcattccggatggccaactgtgcagcgccgggcgggagaagtatcagggcctcgacctggcacgctccgactggacagccacttccttgtcctccggcgtctccttcacatacctctacaaggccaccgccccgcacttgggcttcttcgagttctacgtcaccaaggatggttacgagcccactgagccgctcaaatgggcagacttggaggactcgcccttcatcaacgtcaccgaccccacgcttgtcagcggctcctaccaaatccccggcaccacgccttccggcaagtccggccgccacctcatctacgtcatttggcagcgctccgacagccccgaggccttctactcctgctccgacgtcgacttctcttccgatgccctcatctctctcggctccgcggtactc

SEQ ID NO: 66 - DNA, 657 bp, Bolbitis cladorrhizans
atggggaggtcattgggagctgtggttattacattggtgctgtgcgcgggcggcctgctgagcttagcgagcggccatggcagcatggaggatcccatcagtcgcgtttacaggtgctaccttgagaatccggagagtccgacttcggcggcttgccaagcggcggtggcgctgagtggcaccgaagccttctctggttatgcttggagtgcggtattggccaacgctgcaggccagcaccgccagctcattccagatggccaattgtgcagcgcagggcaggagctgtatgcgggcctagacctgccacgcgccgactggccagccacctccttgtcctctggcgttgccttcacatatctctacaaggccgcgatcccgcacatgggcttcttcgagttctacatcacccgggatggttatgagcccacagagccgctcaagtgggcagatttggaggactcgcccttcctcaacgtcactgaccccccgcttgtcagtagttcctaccagatccctggctccacacctgccggcaagtctggccgccaccttatctatgtcatttggcagcgctccgacagcccccaggccttctactcctgttccgatgtcgactttgttgatgccaccctctctcagctccactccaccacc

SEQ ID NO: 67 - DNA, 660 bp, Dryopteris filix-mas
atgaagaagtcatggggagttgttgtagtagtagtagtagctctagtactgttgtgcctgctgggcacggcaagcggccatggcagcatgcaggaccccatcagtcgtgtctacaactgctacctagagaatcctgagaacccaacgtcggcagcttgcaaagctgtggtggcggtggggggcacgcaaccactctacgattggaatgaggtgaacctggccaacgccgctggccggcaccgtgagctcattcctgatggcaggctgtgcagtgctggccgggacaaatatcggggcctcgacctggctcgcgacgactggccagccacctccttatcctctggtgtcgactacacattcctctaccgcgccactgcccctcacttgggcttcttcgagttctatgtcacccgcgacagctacgaccccacccagccgctcgcatgggcagacctggaggacttgccgttcatcaacgttaccaaccctgccctaaatgctggtgcctaccaaatccccggcaccatgccggccggaaagagcggtcgccacctcatctacgtcatctggcagcgcagcgacagccccgaggcattctactcctgctccgacgtcgacttctcttccgatgccctcatctctctccgctccgcggtactc

SEQ ID NO: 68 - DNA, 654 bp, Pyrrosia lanceolata
atgaggacgaggtcatggggagttgtggcttttatggtagctgtgtgtgccggcgacctgctaggcctcgcgagtgggcatggctccatgggctaccccgtcagtcgcgtcttgaactgcttccttgagaatccggagagccccacgtcggctgcctgcaccgcggcggtggctatgagtggcacccaagccttctacgactggaatgaggtcaatctgccctttgccaatggccagcaccgcgacctcattcctgacggccaactctgcagcgccgggcgcgccaagtatgcaggcctggacctggcacgcgacgactgggaagccacttttttgtcttcggccaccagctacacactcctctacagggtcaccgctcgccacctgggctacttcgagttctacgtcactcgcgatagctacaactccactcagccgctcgcctgggcggacttggaggattcgcccttcatcaacatcaccaaccctaccgttgacagcggctactaccaagtgcctgtcgacacgccttccggcaagactggccgccacctcatctacgtcatttggcagcacaccgacagcctcgaggccttctactcctgctccgacgttgaatttgacgtcgaggtcccctctctccgctccaccacc

SEQ ID NO: 69 - DNA, 654 bp, Athyrium filix-femina
atggggaggtcatgggggggagttgtggctattatggtgttgtgcggctgcctgctgggcgtagcgagcgggcatggcagcatggaggaccccatcagtcgcgtctacaactgctacctggagaatccggagagtcccacgtcggcagcttgccaagcggcggtggcgctgagtgggacccaagcgttctatgattggaatgaggtgaaccagcccttcgccgctggccagtcccgcgagatcattccggatggccaactgtgcagcggcgggcgggagaagtataagggcctcgacctggcacgctccgactggacagccacctccttgtcctccggcgtcgccttcacattcctcttcaaggccaccgccccgcacgcgggcttcttcgaattctacgtcacccaggatggttacgaccccactgagccgctcaaatgggcagacttggaggactcgcccttcatcaacgtcaccgaccccacgcttgtcagcggctcctaccaaatctccggcaccacgcctgccggcaagtccggccgccacctcatctacgtcatttggcagcgctccgacagccccgaggccttctactcctgctccgacgtcgaattcgtcgacgatgccctctctagtgatctccactccaccacc

SEQ ID NO: 70 - DNA, 654 bp, Colysis wrightii (Monstifera)
atggggagagcatgggtagttgtggctattatggtcgccgtgtgcgccagcgggctgctgagcttcgccagtcgcacacggggccatggcagcatgggggaccccatcagtcgagtacttaggtgccgcgaagagaatccggagaatcccacgtcgccagcctgcatcgcggcggtggcgctcagcggcaaacaagccttctacgattggaatgaagtgaatctgcccttcgccgatggccagcaccaaaagctcatccctgacggccaactttgcggcgctgggcgtgacaagtataaaggcctcaacctggcacgtgccgactggctggctacctccttgtctgccggcgccccctacacattcctcttcctggcctccgccccccacctgggctacttcgagttctacgtcactcgggatagttacgaccccactcagccgctcgcatgggcggacttggaggactcgccgttcctcactaccaccacgaccctcgacagcagctcctacataattccaggcaccacgcccgctggcaaaaccggccgccacctcatctacctcatttggcagcgcaccgacagccctgaggccttctactcctgctccgacgtcgactttgaggaggccatctctctttcctccaccacc

SEQ ID NO: 71 - DNA, 657 bp, Coniogramme venusta
atggggaggagctcgtcgtgggagggagtactagtagtagtggtgtgctgcgccagcggcctgctgggcgtagcgagcggccatggcagcatgggcagccccatcagtcgcgtctacaactgccgccaggagaatccggagcgtcccacctcggcagcttgcagagaggcggtgaggattagtgggacccaagcgttctatgattggaatgaggtgaacctgcccgtcgcctctggccggcaccgcgagctcattccggatggcaagctctgcagcgccgggcggactaagtatgcgggcctcgacttggcacgctccgactgggtatccaccgtcttgccctccggcgtcccctacacattcctctacagggtcaccgctcgccacgtgggcttcttcgagttctacgtcacccgggatggttaccagccctctgagcccctcaaatggtcagacttggaagagcctccgttcatcaacgtcaccaatcccacgatgtccggcggcttctatcgaatccccggaaccacgccacccgccaaggccggccgccacctcatctacgtcatttggcagcgctccgacagccccgaggccttctactcctgctccgacgctgtcttcggcgacgccctctctctccagtactcctccacc

SEQ ID NO: 72 - DNA, 651 bp, Platycerium coronarium
atgaggaggtcttggggagttgtggctgttattatgttggcagtgtgcgccgtcggcatgctgggcgtagccagcgggcatggtagcatggaggatcccatcagtcgcgtgtataggtgcttcctggagaacccggagaggcccacgtcagcagcgtgcatcgccgcggtggcgcttagtggcacccaagccttctacgactggaatgaggtaaatctgcccttcgcagctggccgacaccgcgagctcattcctgacggtcagctctgcagcgccgggcgggacaagtataaaggcctcgacctggcacgcgacgactgggtggccacctctttgtcctccggcgtcaactacaccttcctctacaaggccaccgccccccatcggggctacttcgagttctacgtcacccgggatagctacgaccccactgagccgctggcctgggcggacctggaagacacgcccttcatcaacgtcaccgacccggacctcgccagtggctcctaccagatctccagcaccacgccttccggcaagaccggccgccaccttatctacgtcatttggcagcgcaccgacagccccgaggccttctactcctgctccgacatccttttcgacgaggccgtcgctctctactctaccgct

SEQ ID NO: 73 - DNA, 654 bp, Cystopteris bulbifera
atggggagagtcaaccttatggctattttggcgttgtgcgccagcttctgcgccgccctgctgggcgttgccagcggccatggcagcatgcaggaccccatcagtcgcgtctacaactgcttcctggagaacccggagcgtcccacgtcggcagcttgccaagcggcggttgcgctgagtggcacccaagcgttctatgactggaatgaggtgaacctggcgaacgccgatggtcggcatcgcgagctcattccggatggccaactgtgcagcgccgggagggagaagtatcagggcctggacctggcacgcgccgactggacagccacctccttgtcctccggcatctcctacacattcctctacaaggccaccgctccgcacctgggcttcttcgagttctacgtcacccgggatggttacgaccccaccgaggcgctcaaatggtcagacttggaggactcgccgttcctcaacgtcaccaaccccacccttgtcagcggctcctaccaaatccccgttaccacgcctgccgccaagtccggccgccacctgatctacgtcatttggcagcgctccgacagccccgaggccttctactcctgctccgacgtcgacttcgacgatgccctagtctctctccactccaccacc

SEQ ID NO: 74 - DNA, 651 bp, Platycerium ridleyi
atgaggaggtcatggggagttatggctgttattttgttggcggtgtgcgcctgcggcctgctgggcgtagcgagcgggcatggcagcatggaggatcccatcagtcgcgtgtatgggtgctacctggagaatccggagaggcccacgtcggcagcgtgcatcgcggcggtggcgctcagtggcacccaagccttctacgactggaatgaggtgaatcagccctttgcagctggccgacaccgcgagctcattcctgacggtcagctctgcagcggcgggcgggacaagtataaaggcctcgacctggcgcgcgacgactgggaggccacctccttgtcttctggcgccaactacagcttcctcttcaaggccaccgccccccatcggggctacttcgagttctacgtcacccaggatagctacgaccccactgagccgctggcctggggggacctggagagcacgcccttcatcaatgttacggacccggaccttttcagcggctcctaccagatctccagcaccacccctcccggcaagaccggccgccacctcatctacgtcatctggcagcgcaccgacagtcccgaggctttctactcctgctccgacgtccttttcgacgaggccgtcgctctctactctaccgct

SEQ ID NO: 75 - DNA, 645 bp, Dryopteris marginalis
atggggaggtcatggggagttgtggctattattatggtgttgtgcggcagcggcctgctgggcgtagcgagcggccatggcagcatgcaggaccccatcagtcgcgtctacaactgctacctggagaatccggagcgtcccacgtcggcagcttgccaagcggcggtggcgctcagtgggacccaagcgttctatgattggaatgaggtgaaccagcccttcgcggctggccggcaccgcgaaatcattccggatggccaactgtgcagcgccgggcgggagaagtatcggggcctcgacctggcacgctccgactgggtagccacctccttgtcctcgggcgtcaactacacatacctctacaaggccaccgccccgcacttgggcttcttcgagttctacgtcacccaggatggttacaattcctctgagccgctcaaatgggcagacttggaggactcgccgttcatcaacgtcaccaccacgcttgacagcgcctcctaccaaatccccggcaccacgcctgcgggcaagaacggccgccacctcatctacgtcatttggcagcgctccgacagccccgaggccttctactcctgctccgacgtcgacttcgccgatgccctctctctccactccaccacc

SEQ ID NO: 76 - DNA, 648 bp, Microsorum musifolium (Blume)
atgagaaggtcatggggagttctggctatcgtgatggccgtgtgcgcaagcggcctgtttggcgtcgcgagtggccatggctctatggagcaccccattagtcgcgtctatcaatgctaccgcgagggtccggaaaatcccaagtcgccagcctgcatcgcggcaaaggggcttagcggcgctcaagccttctacgattggaatgaagtgaatcagcccttcgccgatggccgccaccaggagatcatccatgacggccatctttgcagcggcgggcgcgacaagtatagaggcctcgacctgccacgtgccgactgggtggctacctctttgtctgccggaaaaccctacacattcctctaccgggccaccgcccaccacctgggctacttcgagttctacgtcactcgggacggctacgaccccactaagccgctcgcatgggcggacttggaggactcgccgtttatcaatgtcaccaacccgaccctcgtcagcggcagctaccgaattccacacaccacgcccgccagcaaaactggccggcacctcatctacgtcatttggcagcgcaccgacagcttcgaggctttctactcctgctccgacgtcgtctttgatgaggccctctctctttcctccaccatc

SEQ ID NO: 77 - DNA, 648 bp, Elaphoglossum sp.
atgcggagatcatgggaagttgtggctctaattatggtggtgtgcgcctgcggcctgctgggcgtagcgagtggccatggcagcatggaggaccccatcagtcgtgtctacaggtgctacctcgagggagtggagaatcccacgtcggcagcctgcatagcggccattgaggtgagtggcaagcaagccttctacgactggaatgaagtgaatcagcccttggccgctggccggcaccgcgaaatcattcctgacggcgagctgtgcagcggcgggcgggagaagtataaaggcctcgacttggcacgcgccgactggttagccacctccttgtcttcgggtgtcgactacacattcctctacaaagccaccgccgaacacaagggctacttcgagttctacgtcactcaggatagttacgaccccacggagcctctcaaatggtcggacctggaggacacgcccttcattaacgtcacccaacccttgcttgtcagcggctcctaccaaattcccggcaccacgccttccggcaaaaccggccgccacctcatctacgtcatctggcagcgcaccgatagcgccgaagccttctactcctgctccgatgtcaactttgacgacgccctccctatctactctgccacc

SEQ ID NO: 78 - DNA, 645 bp, Nephrolepis exaltata (Tiger Fern)
atggggaggtcatggggagttgcggctattgtagtggcggtgtgcgccagcggcctgttgagcgtagtgagcggccatggaagcatgcaggaccccatcagtcgcgtctatgcatgctacctagagaatccggagcgtcccacgtcagcagcttgccaggcggcagtggcattgagtgggacgcaagccttctatgattggaatgaggtgaacctgcccaatgccgctggccggcaccgcgaactcattccggatggtcagttgtgcagtgctgggcgggccaagtatcagggcctcgaccaggctcgcaacgattggccacacaccgacttgatctccggcgtcgccttcacattcaactacagggccaccgccccacacttgggcatcttcgagttctatgtcactcgggatgggtacgatgccacccagcccctcaaatgggcagatctggaggactcgcctttcctcaccgccaccagcacgcttgccccctcctcctaccagtggcccggcaccactcccagtggcaagtctggccgccacctcatctacgtcatttggcagcgcaccgacagccccgaggccttctactcctgctccgacgtcgagttcgtcgatgccgtctctctccactccaccacc

SEQ ID NO: 79 - DNA, 642 bp, Dryopteris lepidopoda
atggggaggtcatggggagttgtggctattatggtgttgtgcggcagcggcctgctgggcgtggcgagcggccatggcagcatggaggaccccatcagtcgcgtctacaactgctacctggagaatccggagcgtcccacgtcggcagcttgccaagcggcggtggcgctgagtgggacccaagcgttctatgattggaatgaggtgaaccagcccttcgcggctggccggcaccgcgaaatcattccggatggccaactgtgcagcggcgggcgggagaagtatcggggcctggacctggcacgctccgactgggaagccacctccttgtcctccggcgtcagctacacatacctctacaaggccaccgccccgcacttgggcttcttcgagttctacgtcacccaggatggttacaactcctctgagccgctcgaatgggcagacttggaggactcaccgttcatcaacgtcaccaccacgcttgacagcgcctcctaccaaatccccggtaccacgcctgccggcaagaccggccgccacctcatctacgtcatttggcagcgctccgacagccccgaggcattctactcctgctccgacgtcgacttcgtcgatgccctctctctccactccaccacc

SEQ ID NO: 80 - DNA, 642 bp, Polystichum lepidocaulon
atgggcaggtcatggggagttgtggctattatggtgttgtttgccagcgctagcggcctgctgggcgtagcgaacggccatggctccatgggcaaccccatcagtcgcgtctacaactgcaggctggagaatccggagagacccacgtcggcagcttgcatagcggcggtggcgctgagtggcacctatgattggagtgaggtgaacctgcccaacgccaatggccggcaccgcgagctcattccggatggcaaactgtgcagcgccgggcgggacaagtataagggcctcgacctggctcgctccgactggacagccaccaacttgtcctccggcgtcgcctacacattcctctacagggtcaccgccgagcacagggggttcttcgagttctacgtcaccgtggatgattacgaacccactgagctgctcaaatgggaagacttggaggaaacgccgttcctcaacgtgagtgaccccacggtcgtaggcaacaactacgaaatctccggcaccacgcctgccagcaagactggccgccacctcatctacgtcatttggcagcgctccgacagccccgaggccttctactcctgctccgacgtcgacttcgtcgataccctgtctctccactccaccacc

SEQ ID NO: 81 - DNA, 645 bp, Polystichum acrostichoides
atggggaggtcatggggagttgtggctattatggtgttgtgcgctagcggcctgctgggtgtagcgagcggccatggcagcatgaacgaccccatcagccgcgtctacaactgccgtctggagaatccggagagtcccacgtcagcagcttgcatagcggcggtggcgctgagtgggacccaagcgttctatgattggaatgaggtgaacctgcccgacgtcaatggccggcaccgccagctcattccggatggcaaattgtgcagcgccgggcgggacaagtataagggcctcgacctggcacgctccgactgggtagccaccaacttgtcctccggcgtcgccttcacattcctctacagggtcaccgcccagcacaggggcttcttcgagttctacgtcaccgtggatgattacgaccccactgagctgctcaaatgggaagacttggaggaaacgccgttcatgaacgtcaccgaccccacggttgtaggcgtcaattacgaaatccccggcaccacgcctgccaataagaccggccgccatctcatctatgtcatttggcagcgctccgacagccccgaggccttctactcctgctccgacgttgacttcgtcgatgccgtgtctctccactccaccacc

SEQ ID NO: 82 - DNA, 645 bp, Davallia tyermannii
atggggaggtcatggggagttgtggctattatggtgatgtacattggtggcctgctaagcatagcaagcggccatggcagcatggaggaccccatcagccgcgtctataggtgctacttggagaatccggagagtcccacatcggcagcttgccaagcggcagtggcagtgagtggggcccaagccttctacgattggaatgaggtgaacattgctgacgccaatggccgacaccgggagctcatttctgatggccaactatgtagcgcaaatcggagtaagtatgcgggcctcgacctggcacgcgcagattggctaggcaccaccttgtcctcgggcgcctccttcacatttgcctacaaggccaccgcgccgcacttgggcttctttgagttctacgtcacccgggatggttacgagcccaccgacccgctcaaatgggcagacttggaggactcgcccttcatcaacgtcaccaaccccacacttgataatggcgcctaccagatctccggcaccacgcctgccggtaagtcggggcgtcatctgatctacgtcatttggcagcgctctgatagcccagaggcattctattcgtgctccgacgtcgactttgtcgatgctctctctctccactctaccacc

SEQ ID NO: 83 - DNA, 645 bp, Polystichum polyblepharum (C.)
atggggaggtcatggggagttgtggctattatggtgttgtgcgctagcggcctgctcggcgtagcgagcggccatggcaccatgaatgaccccatcagccgcgtctacaactgccgcctggagaatccggagagtcccacgtcagcagcttgcatagcggcggtggcgctgagtgggacccaagcgttctatgattggaatgaggtgaacctgcccaacgccgctggcaggcaccgagagctcattccggatggcaaactgtgcagcgccgggcgggacaagtataagggcctcgacctcgcacgctccgactgggtagccaccaacttgtcctccggcgtcgccttcacattcctctacagggtcaccgcccagcacaggggcttcttcgagttctacgtcaccgtggatgattacgaccccactgagctgctcaaatgggaagacttggaggaaacaccgttcatgaatgtcaccgaccccacggttgtaggcgtcaactacgaaatggccggcaccacgcctgccaacaagaccggccgccatctcatctatgtcatttggcagcgctccgacagccccgaggccttctactcctgctccgacgtcgacttcgtcgatgccgtgtctctccactccagcacc

SEQ ID NO: 84 - DNA, 648 bp, Lecanopteris sinuosa
atgatgaggtcatggggagttgcggcaattatgatggccgtctgcgccagtggcctgctgggcgttgcaagtgggcatggcagcatggcggaccccatcagtcgggtgtacaggtgccgcctcgagaatcccgaaaggcccacgtcgccagcctgcattgcggcggtggcgcttagcggcactcaagccttctacgactggaatgaagtgaatcttcccttcgctgctggccgccaccgccagctcatccccgacggacaactttgcagcgccgggcggaacaagtataaaggcctcgacctcgcacgcgccgactggctagccacctccctgtctcccggcgccaattacacattcctctaccgggcgaccgccccccacgcgggctactttgagttctacgtcactcgtgatagctacgaccccactgagcagctcgcttgggcggacttggaagactcgccgttcatcaccatcaccaacccgacccttgtcaacggctactaccagattcccaacaccgtccctgccggcaaaactggccgtcaccttatctacgtcatttggcaacgcacagacagtcccgaagccttctactcctgctccgacgtcgactttgacgatgccctccgtctccactactccacc

SEQ ID NO: 85 - DNA, 645 bp, Aglaomorpha splendens
atgaggaggtcatggggagtggtggtgattttggtggtgtgcgtctgcggcctgctgggcgtggcgagtgggcatggctccatgggggaccccatcagtcgcgtctatgggtgccgccttgagaatccggagagtcccacgtcggcagcctgcatagcggcggtggcggtgagtggcacccaagccttctacgattggaatgaggtgaatcagcccaacgccaatggccggcaccgcgagatcattccagatggcgaactgtgcagcgccgggcgggtaaaatatgcaggcctcgatctggcacgcgacgactgggtagccacctccttgtcttctggcgtcaactacacattcctcttcgtagccaccgccccccacttgggctacttcgagttctacgtcactcaggatagctacgaccccacccagccgctcaaatggtcggacttggaggccaccccgttcatcaacgtcaccgatcccacgcttcttaacggctcctaccaaattcccagctccacgccctccggcaaaaccggccgccacctcatctacgtcatttggcagcgcactgacagccctgaggccttctactcctgctccgacgtcgactttgatgtggccctccctctttactcctccacc

SEQ ID NO: 86 - DNA, 645 bp, Nephrolepis exaltata; identical to SEQ ID NO: 78

SEQ ID NO: 87 - DNA, 645 bp, Aglaomorpha splendens; identical to SEQ ID NO: 85

SEQ ID NO: 88 - DNA, 648 bp, Polypodium formosanum
atgaagagatcgtggggagttgctgctattgtgatggccctgagcacttgcggcttgataggcgtagcaagtggccatggctccatgggagaccccatcagtcgcgtctataggtgctaccgagagaatccggagcgtcccacgtcgccagcctgcattgcggcggtggcgctgagtggcaagcaagccttctacgattggaatgcggtgaatctgttcaacgccaacggtcgacaccgcgagctcattcctgacggccagctctgcagtgccgggcgggccaagtataaaggccttgacctcccacgcgccgattggctagccacctccttatcctccggcgtcaacttcacattcctctacagggtcaccgcccgccacctgggctatttcgagttctacgtcactcgcgatggctacgaccccagtgaaccgctcgcatgggcggacttggaggactcgccgttcatcaaaatcaccaacccatccgttgtcagcaactcctatgtaattcccggcatcacgcctgccggcaaaactggccgccaccttatttacgtcatttggcagcgcaccgacagccaggaggccttctactcctgctccgacatcgactttgacgaggccgtccctctctactccaccacc

SEQ ID NO: 89 - DNA, 642 bp, Nephrolepis obliterata (Sunjest)
atggggaggtcatggggagttgtggctattatggtggtgtgcgcttgcggcctattgagcgtagtgaggggccatggaagcatggaggaccccattagtcgcgtctatgggtgctacctagagaatccagagagtcccaagtcagcagcttgccaagcggcagtggcattgagtgggacccaagcgttctatgattggaatgaggtgaacttgcccgatgttgctggccggcaccgcgcagtcattccggatggccaattgtgcagtgctgggcgggctaagtatcagggcctcaacttggctcgcgccgattggccagccacctccttgacctcaggcgtgtccttcacatacctctacaaggtcaccgcaaaacacttgggcttctttgagttctatgtcactcaagatggttacgatcccaccgaaccgctcaaatgggcagacttggaggacttgcctttcatgaacgtcaccagcacgtttgacgatgagtcctaccaaatgtctggcaccactcctagtggcaaggctggccgccacctcatctacgtcatttggcagcgcagcgacagccctgaggccttctactcctgctccgatgtcgacttcgtcgatgccgtctctctccgctccaccacc

SEQ ID NO: 90 - DNA, 645 bp, Deparia acrostichoides
atggggaggtcatggggagttgtggctattatggtgttgtgcgccagcggtctgctgggcgtagcgagcggccatggcagcatggagggccccatcagtcgcgtcctcaactgctacctggagaatccggagagacccacgtcgggagcttgcatagcggcggtggcgctgggtgggacacaaccgttttatgattggaatgaggtgaacctggccgatgccgatggccggcaccgcgagctcattccggatggccaactgtgcagcgccggacgggagaagtttaagggcctcgacctggcacgctccgactggccagccacctccttgtcctccggcgtcgccttcacatacctctacaaggccaccgccccacacgctggcttcttcgagttctacgtcacccgggatggttacaagcccactgagccgctcaaatgggcagacttggaggagccaccgttcatcaacgtcaccgaccccaagcttgtcagcggctcctaccaaatccccggcaccacgcctgccggcaaggctggccgccacctcatctacgtcatttggcagcgctccgacagccccgaggccttctactcctgctccgacgtcgacttcgtcgaagccctctctctccactccaccacc

SEQ ID NO: 91 - DNA, 648 bp, Aglaomorpha sp. (Roberts)
atgaggaggtcatggccgggagtggtggcgattatggtggtgtgtgcctgcggcctgctgggcgtggcgagtggccatggctccatgcaggaccccatcagtcgggtctataggtgccgccttgagaatccggagcggcccacgtcggcagcctgcatagcggcggtggcgctgagtggcacccaagccttctacgactggaatgaggtgaatcagcccttcgccaatggccgccaccgcgagatcattccggacggccaactgtgcagcgccgggcgggcaaagtatagaggcctcgacctggcacgcgccgactggctagccccctccttgtcttctggcgtcgactacacatttctctacatagccactgccccccatttgggctacttcgagttctacatcactcgggatagctacgaccccaccgagccgctcaaatggtcggacttggaggactctccgttcatcaacgtcaccaacccctcgcttgtcagcggctcctaccaaattcccggcaccacgccctccaacaaaaccggccgccacctcatgtacgtcatttggcagcgcaccgacagccccgaggccttctacgcctgctctgacgtcgactttgatgtggccctccctctctactccaccact

SEQ ID NO: 92 - DNA, 642 bp, Nephrolepis obliterata; identical to SEQ ID NO: 89

SEQ ID NO: 93 - DNA, 645 bp, Polypodium attenuatum (Falax)
atggggaagggatgggaagttgtgggtataatggtggtgtgcgcctgcggcctgctgggcgtggccagtgggcatggcaccatggaggaccccatcagtcgcgtctacaggtgccgccttgagaatccggagcgacccacgtcgccagcctgcatagcggcggtggcgctgagcggcactcaagccttctacgattggaatgaggtgaatctgcccttcgccgccggccggcaccgcgagatcattcccgacggccagctgtgcagcgccgggcgcgccaagtatagggggctggatctggcacgcgatgactggctagccacctccttgtcttccggcgtcgactacacattcgtctacagagtcaccgcgccccaccgtggctacttcgagttctacgtcactcgggacacctacgaccccactgagcccctcaaatggtcggacttggaggagccccccttcatcaacgttacccaaccctcgcttgtcagcggctcctaccagattcccggcgccacgcctaccggtaagaccggccgccacctcatctacgtcatctggcagcgcactgacagccccgaagccttttactcctgttccgacgtcgactttggcgaggctctccgtctcgacgccaccgcc

SEQ ID NO: 94 - DNA, 645 bp, Arachniodes simplicior (variegata)
atggggaggtcatggggagttgtggctattatagtgttgtgcgccagcggcctgctgggcgtagcgagcggccatggcagcatggaggaccccatcagtcgcgtctacaactgcttcctggagggtccggagaatcccacgtcggacgcttgcatagcagctgtggcgctgagtgggacccaagcgttctatgattggacggaggtgaacctggccgacgccgatggccatcaccgcgagctcattccggatggccaactgtgcagcgccgggcgggacaagtacaagggcctcgacctcgcacgctccgactggacagccacgtcattgtcctccggcgtcgactacacattcctcttcaaggccaccgccccgcacttgggctccttcgagttctacgtcactgtggatggttacgagcccactgagccgctcaaatgggcagacttggaggcaacgccattcatcaacgtcaccgaccccacgcttgacagcggctcctaccaaatccctggtaccacacctgccggcaagaccggccgccacctcatctacgtgatttggcagcgctccgacagtgccgaggccttctactcctgctccgacgtcgacttcactgatgccctctctctccactccaccacc

SEQ ID NO: 95 - DNA, 648 bp, Campyloneurum angustifolium
atgaggaggtcatgggaggttgtggggatgatggtgctgtgcgcctgcggcctgctgggtgtagcgagcggccatggcagcatggaggaccccatcagtcgcgtctataggtgccgccttgagggtccggagaggccaacgtcgccggcctgcatagcggcggtggcggtgaatggcactcaggccttctacgactggaatgaggtgaatcagcccttcgccgctgggcggcaccgtgagatcattcccgacggccagctctgcagcgccgggcgggacaagtataaagggttggacctggcgcgcgccgactggctagccgtctccttgtcttccggcgccgactacacattcctctacctagccaccgccacccacaggggctacttcgagttctacgtcactcgggatagctacgatcccactgagccgctcaaatggtcggacttggaggactccccgttcatcaacgtcacggatcccacagaagtcggccccgtgtaccaaattcccggcaccacgcctgccggcaaaactggccgccacctcatctacgtcatttggcagcgcaccgacagccccgaagccttctactcctgctccgacgtcgactttggcgagtctctctccctctactccgtcaccgag

SEQ ID NO: 96 - DNA, 645 bp, Colysis wrightii (Ching)
atgaggaagtcattggaagttgtggctattatggtggccgtgtgcgccagcggcctactgggcgtcgcgagtggccatggcaccatgctggaccccatcagtcgcgtctataggtgctacctcgagaatccggagcgtcccacgtccccagcctgcatcgcggcggtggcgctcagcggcaaacaagccttctacgattggaatgaagtgaatctgcccttcgcggctggccgtcaccgcgagctcatccctgacggccaactttgcagcgctgggcgggacaagtataaaggcctcgatcaggcacgtgacgactggctggctacctccttgccttccggcgccaactacatattccgctttgaggtcaccgccgtccaccgtggctacttcgagttttacgtcactcgcgatggttacgaccccactcagccgctcgcatgggcggacttggaggactcgccgttcctcactaccaccacgaccctcgacagcagctcctacataattccaggcaccacgcccgctggcaaaaccggccgccacctcatctacctcatttggcagcgcaccgacagccctgaggccttctactcctgctccgacgtcgactttgaggaggccatctctctttcctccaccacc

SEQ ID NO: 97 - DNA, 645 bp, Colysis wrightii (Ching)
atggggaggtcatgggtagttgtggctattatggtcaccgtgtgcgccagcggcctgctgggcttcgccagtggccatggcagcatgggggaccccatcagtcgagtacttaggtgccgcgaagagaatccggagaatcccacgtcgccagcctgcatcgcggcggtggcgctcagcggcaaacaagccttctacgattggaatgaagtgaatctgcccttcgcggctggccgtcaccgcgagctcatccctgacggccaactttgcagcgctgggcgggccaagtataaaggcctcgatctggcacgtgacgactggctggctacccccttgccttccggcgccgcctacacattccgctatcgggtcaccgccgcccaccgtggctacttcgagttctacgtcactcgggatggttacgaccccactcagccgctcgcatgggcggacttggaggactcgccgttcctcactaccaccacgaccctcgacagcagctcctacataattccaggcaccacgcccgctggcaaaaccggccgccacctcatctacctcatttggcagcgcaccgacagccctgaggccttctactcctgctccgacgtcgactttgaggaggccatctctctttcctccaccacc

SEQ ID NO: 98 - DNA, 648 bp, Platycerium elephantotis
atgaggaggtcatggggggttgtggctgttatgttggcgatctgcgccagcggcctgctgggcgtagcgagcggccatggcagcatgctggatcccatcagtcgcgtgtatacgtgctatttggagaatccggagaggcccacgtcggcagcgtgcatcgcggcggtggcggtcagtggctcccaagcgttctacgattggaatgaggtgaatctggccgatgcagatggccagcaccgccagctcattcctgacggcaagctctgcagcgccgggcgggaaaagtacagaggcctcgacctcgcacgcgatgattggcctgccacctccttgtcttctggagtcaattacaccttcctctacagggccaccgccccccacctgggcttcttcgagttctacgtcacccgtgatagctacgaccccactcagcccctggcctgggcggacctggaagaccccccctttatcaacatcaccgacccaacccttgccagcggctcctaccagattgttaacaccacgccttccaacaagaccggccgccacctcatctacgtcatctggcagcgtactgacagccccgaggccttctactcctgctccgacgtcgacttcgacgaagatgactctcttctctccgcagtt

SEQ ID NO: 99 - DNA, 645 bp, Platycerium madagascariense
atgaggaggtcgtggggggttgtggctgttatcttggcaatgtgcgccggtagcctgctcggcgtagcaagcggccatggtagcatggaggatcccatcagtcgcgtgtatgcgtgcttcctggagaatccggagagacccacgtcggcagcatgcatcgcggcggtggcgctgagtggcacccaagccttctacgactggaatgaggtgaatcagcccaatgccgctggcaaccacacaatcattcccgacggccagctctgcagtgccgggcgggagaagtacaaaggcctcgacctcccacgcgccgactggtctgccatctccttgtcttccggcgtaaactacaccttcctttacaaggctaccgccccccaccggggctactttgagttctacgtcacccgtgatagctacgaccccactgagccccttgcctgggcggacctggaagacacccccttcatcaacatcaccgacccagaccttgtcagcggctcctaccggattgctaacaccaccccttccggcaagaccggccgccacctcatctacgtcatttggcagcgtaccgacagccccgaggccttctactcctgctccgacgtcgtcttcgacgaggatgtctctctcgtctccgcagct

SEQ ID NO: 100 - DNA, 648 bp, Microsorum musifolium (Blume)
atgagaaggtcatggggagttctggctatcgtggtggccgtgtgcgcaagcggcctgtttggcgtcgcgagtggccatggctctatggagcaccccattagtcgcgtctatcaatgctaccgcgagggtccggaaaatcccaagtcgccagcctgcatcgcggcaaaggggcttagcggcgctcaagccttctacgattggaatgaagtgaatcagcccttcgccgatggccgccaccaggagatcatccatgacggccatctttgcagcggcgggcgcgacaagtatagaggcctcgacctgccacgtgccgactgggtggctacctctttgtctgccggaaaaccctacacattcctctaccgtgccaccgccccccacttgggctacttccagttttacgtcactcgcgacggctacaaccccactaagccgctcgcatgggcggacttggaggactcgccgtttatcaatgtcaccaacccgaccctcgtcagcggcagctaccgaattccacacaccacgcccgccagcaaaactggccggcacctcatctacgtcatttggcagcgcaccgacagccccgaagccttctactcctgctcggacgtcgtctttgatgaagccctctctctctcctccaccatc

SEQ ID NO: 101 - DNA, 657 bp, Lygodium flexuosum
atggggagctggcagtggggatcagtgaatgtggccattgttgtttttatgatgttgtgcggcgtagcgagcggccatggcaccatgggggaccccatcagtcgcgtctacaggtgctaccttgagaatccggagaggcccacgtcggcagcttgccaagcggcggtggcgctgagtgggacccaagccttctacgactggaatgaggtaaacctgcccaacgccgctggccggcaccgccagctcattccggatggccaactgtgcagcgccgggcgggccaagtatcagggcctcgacctggcacgcgccgactggctagccgccagcctgtcctccggcgtctcctacacattcctctacagggtcaccgcccagcaccgtggcttcttcgagttctacgtcacccgggatggttacgagcccactgagccgctcaaatggtcagacttggaggagtcgccgttcatcaacgtcaccgaccccacggctgtcagcggctcctaccagatccccggcaccacgcctgccggcaagtccggccgccacctcatctacgtcatttggcagcgctccgacagccccgaggccttctactcctgctccgacgtcgacttcgacgtcgagggcgccgccgtctctctccgctctaccacc

SEQ ID NO: 102 - DNA, 645 bp, Polystichum polyblepharum
atgaacaggtcatggggagttgtggctattatggtgctgtgcgctagcggcctgctcggcgtagcgagcggccatggcaccatgaatgaccccatcagccgtgtctacaactgccgcctggagaatccggagagtcccacgtcagcagcttgcatagcggcggtggcgctgagtgggacccaagcgttctatgattggaatgaggtgaacctggccaacgtcgctggccggcaccgcgagctcattccggatggcaaactgtgcagcgccgggcgggacaagtataagggcctcgacctcgcacgctccgactgggtagccaccaacttgtcctccggcgtcgccttcacattcctctacagggtcaccgcccagcacaggggcttcttcgagttctacgtcaccgtggatgattacgaccccactgagctgctcaaatgggaagacttggaggaaacgccgttcatgaatgtcaccgaccccacgcttgtaggcctcaactacgaaatgcccggcaccacgcctgccaacaagaccggccgccatctcatctatgtcatttggcagcgctccgacagccccgaggccttctactcctgctccgacgtcgacttcgtcgatgccgtgtctctccactccagcacc

SEQ ID NO: 103 - DNA, 654 bp, Diplazium pycnocarpon
atggggaagtcatggggagttgtggctattatattggtgttgtgcgccagcggcctgctgggtgtagcgagcggccatggcagcatggcggaccccatcagtcgcatttacaactgcagacaggagaatccggagcgtcccacgtcggcagcttgccaagcggcagtggcgctgagtggaacccaagcgttctatgattggaatgaggtgaaccagcccaacgccgctggccggcaccgcgagatcattccggatggccaactgtgcagcgccgggcggtacaagtatcggggcctcgacctggcaagcgccgactggcagtggcctgccacctccttgtcctccggcgtctccttcacataccgctacagggccaccgccgcgcactacggctacttccagttctatatcacccgggatggttaccagcccactcagccgctcaaatgggcagacttggagcagctgccattccttaccgtctacaaccccacgcttgtcaacggcttctacgaaatgcaggggaccacgcctgctggcaagaccggccgccacctcatctatgtcatctggcagcgctccgacagccccgaggccttctactcctgctccgacgtcgacttcgtgggtgccctctctctccattccaccacc

SEQ ID NO: 104 - DNA, 648 bp, Polystichum braunii
atggggaggtcatggggagttgtggctattatggtgttgtgtgctagcggcctgctgggcgcagcgagcggccatggcaccatgtacgacccattcagccgcgtctacaactgccgcttccgggagaatccggagcgtcccacgtcagcagcttgcatagcggcggtggcgttgagtgggacccaagcgttctatgattggaatgaggtgaacctggccaacgccgctggccggcaccgcgagctcattccggatggcaaactgtgcagcgccgggcgggacaagtataagggcctcgacctggcacgctccgactgggtagccaccaacttgtcctccggcgtcgccttcacattcctctacagggtcaccgcccagcacaggggcttcttcgagttctacgtcaccgtggatgattacgaccccactgagtcgctcaaatgggaagacttggaggaaacgccgttcctcaacgtcaccgaccccacggttgtaggcgtcaactaccaaatctccggcaccacgcctgccagcaagaccggccgccacctcatctacgttatatggcagcgctccgatagccctgaggccttctactcctgctccgacgtcgacttcgtcgatgccctgtctctccaatccaccacc

SEQ ID NO: 105 - DNA, 645 bp, Platycerium hillii
atggggaagccgtggagagtggtggtggccattgtggtggtgtgcgccagcggcctgctgggcgtagcgagcggccatggcagcatgggtgaacccatcagtcgcgtctataattgctacctggagaatccggagagacccacgtcggcagcgtgcatcgcggcggtggcgcttagtggcacccaagccttctacgactggaatgaggtgaacctgcccttcgccgctggccggcaccgcgagctcattcctgacggccagctctgcagcgccgggcgggacaagtataaaggcctggacctggcacgcgccgactgggttgccacctccttgtcttcgggcgtcagctacaccttcctctacagggttaccgccccccaccggggctactttgagttctacgtcaccaaggatagctacgaccccactgagccgctggcctgggcagacctggaggacacgcccttcattaacatcaccgacccgaccattgtcagcggctcttaccagatctccagcaccacgccttccgacaagaccggccgccacctcatctacgtcatttggcagcgcaccgacagccctgaggccttctactcctgctccgatatcgactttgacgacaccctccccctacactccacc

SEQ ID NO: 106 - DNA, 681 bp, Drynaria rigidula (whitei)
atggggaggacgtactcatggggggctgtggctgttatggtggtgctgtgcgccagcggcctgctgggcatagcgagcggccatggcagcatggacagccccatcagtcgcgtctaccggtgctatctagagaatccggagaatcccacgtcggcagcctgccaagcggcggtggcgctgagtgggacccaagccttctacgactggaatgaggtgaacatcgccgacgctgcgggccgccaccgcgagctcattccggatggccaactgtgcagcgccgggcgggaaaagtatcaaggtctcgacctggcacgcgccgactggctagccgactccttgtcctccggcgtctccttcactttcctctacaaggctactgccgcgcacttgggcttcttcgagttctacgtcacccgggatgcctacgaccccactgagccgctcaaatgggcagacctggaggactcgcccttcctcaacgtcaccgaccccacgcttgtcagcggctactaccagatccctggcaccacgcctgccggcaagtccggccgccacctcctctacgtcatctggcagcgctccgacagccccgaggccttctactcctgctccgacgtcgactttgacgacgatgccgctgccgcccagcacatgataatctctctccgccactccaccacc

SEQ ID NO: 107 - DNA, 687 bp, Adiantum monocolor; identical to SEQ ID NO: 44

SEQ ID NO: 108 - DNA, 669 bp, Pellaea rotundifolia
atgcagaggtcatgcatgtggggggaatccgtagtggctattatgtgcatggtgttgggccttctgggcgacgtagcgagcggccatggcagcatggccagccccatcagtcgcgtcttcaactgctacctcgagaatccagagagtcccacctcggaagcttgcaaagcggctgtggaggagagtggcacccaagctttctatgattgggctgaggtgagcctgcccaacgccgctggacgccaccgcgagctcattccggatggccaactctgcagcgccgggctggccaagtatgcgggcctcgacctggcgcgcgccgactggacagccacctccttgacctccaacatctcctacacgttcatcttcgaggccaccgccggcccgcacttgggctccttcgagttctacgtcaccaatgatgattacgagcccgctgaggcgctcaactgggcagacttggaggacactccgttcatcatcgtcaccaaccccacgcttgtgagcggctcctacctcatcccgggcactacgcctgccggcaagaccggccgccacatcatctacgtcatttggcagcgctccgacagccccgaggctttctactcctgctccgacatcgacttcgtggaggaggatcccgtggtccctctccactctaccacc

SEQ ID NO: 109 - DNA, 645 bp, Platycerium bifurcatum
atggggaagccgtggagagtggtggtggccattgtggtggtgtgcgccagcggcctgctgggcgtagcgagcggccatggcagcatgggtgaacccatcagtcgcgtctataattgctacctggagaatccggagagacccacgtcggcagcgtgcatcgcggcggtggcgcttagtggcacccaagccttctacgactggaatgaggtgaacctgcccttcgccgctggccggcaccgcgagctcattcctgacggccagctctgcagcgccgggcgggacaagtataaaggcctggacctggcacgcgccgactgggttgccacctccctgtcttcgggcgtcagctacaccttcctctacagggccaccgccccccaccagggctactttgagttctacgtcaccaaggatagctacgaccccactgagccgctggcctgggcggacctggaggacacgcccttcattaacatcaccgatccgacccttgtcagcggctcttaccagatccccagcaccacgccttccgacaagaccggccgccacctcatctacgtcatttggcagcgcaccgacagccctgaggccttctactcctgctccgatatcgactttgacgacaccctccccctacactccacc

SEQ ID NO: 110 - DNA, 648 bp, Microsorum punctatum
atgaggaggtcatggggagttctggctattgtggtggccgtgtgcgcaagcggcctgtttggcgtcgcgagtggtcatggctccatggaggaccccattagtcgcgtctatcaatgctacgacgagggtccggaaaatcccaagtcgccagcctgcatcgcggcggtggggcttagcggcgctcaagccttctacgattggaatgaagtgaatcagcccttcgccgctggccagcacaaggagatcatccatgacggccatctttgcagcggcgggcgcgacaagtatagaggcctcgacctgccacgtgccgactgggtggctacctctttgtctgccggcgcaccctacacattcctctaccgcgccaccgcccaccacctgggctacttcgagttctacgtcactcgggacggctacgaccccactaagccgctcgcatgggcggacttggaggactcgccgtttatcaatgtcaccaacccgcccctcgtcagcggcagctaccgaattccagacaccacgcccgccctcaaaactggccggcacctcatctacgtcatttggcagcgcaccgacagccccgaagccttctactcctgctcggacgtcgtctttgctgaggccctctctctttcctccaccacc

SEQ ID NO: 111 - DNA, 651 bp, Woodwardia fimbriata
atggggaggtcaatatggggagttgtggctatgatggtgttgtgcgccagcggcctgctgcgcatagcgagcgggcatggcagcatggagaaccccatcagtcgcgtctacaactgctatctggagggtccggagaatcccaagtcggcagcttgcaaagcggcggtggcggcgagtgggacccaagcgttctatgattggaatgaggtgaacctggccaacgccgctggccgccaccgcgagctcattccggatggccaactgtgcagcgccgggcggcagaagtatcagggcctcgacctcgtacgctccgactggccagccacctccttgtcctccggcgtccccttcacattcctctacaggatcaccgcccagcacttgggcttcttcgagttctacgtcacccgcgatggttaccagcccactgcggcgctcacttgggcagacttggaggactccccgttcatgaacgtcaccggcgaccccacgtttatcaccggctcctgggaaatccccggcacctcgcctgccggcaagtctggccgccaccttatctacgtcatctggcagcgctccgacagccccgaggccttctacgcctgctgcgacgtcgacttcgtcgacgccctctctctccactccaccact

SEQ ID NO: 112 - DNA, 639 bp, Dryopteris celsa
atggggaggtcatcattgggagttgtggctattatggtgttgtgcctggtgggcgtagcgagcggtcatggcagcatgcaggaccccatcagtcgcgtctacaactgctacctcgagaatccggagagtcccacgtcggcagcttgccaagcggcggtggcgctgagtggcacccaagcgttctatgactggaatgaggtgaaccagcccgaagccgatggtcggtcccgcgaaatcattccggatggccaactgtgcagcggcgggcgggagaagtatcagggcctggacctggcgcgctccgactgggaagccaccaccttgtcctccagcgtcaactacacattcctctacaaggccacagccccgcacttgggcttcttcgagttctacgtcacccaggatggttacgatcccactgaggtgctcaaatgggcagatctggaggactcgccgttcctcaacgtcaccgaccccacgcttgacagcggcgcctaccaaatccccggcaccacgcctgccggtaagaccggccgccacctcatctacgtcatttggcagcgctccgacagccccgaggccttctactcctgctccgacgtcgacttccccgatgccctctctctccactccaccacc

SEQ ID NO: 113 - DNA, 648 bp, Campyloneurum angustifolium
atgaggaggtcatgggaggttgtggggatgatggtgctgtgcgcctgcggcctgctgggtgtagcgagcggccatggcagcatggaggaccccatcagtcgcgtctataggtgccgccttgagaatccggagagacccacgtcaccagcttgcagagcggcggtggcgttgagtggcactcaggccttctacgactggaatgaggtgaatcagcccttcgccgctgggcggcaccgtgagatcattcccgacggccagctctgcagcgccgggcgggacaagtataaagggttggacctggcgcgcgccgactggctagccgtctccttgtcttccggcgccgactacacattcctctacctagccaccgccacccacaggggctacttcgagttctacgtcactcgggatagctacgatcccactgagccgctcaaatggtcggacttggaggactccccgttcatcaacgtcacggatcccacagaagtcggccccgtgtaccaaattcccggcaccacgcctgccggcaaaactggccgccacctcatctacgtcatttggcagcgcaccgacagccccgaagccttctactcctgctccgacgtcgactttggcgagtctctctccctctactccgtcaccgag

SEQ ID NO: 114 - DNA, 654 bp, Onoclea sensibilis
atggggaggtcatggggagtggtgcaggctataattatggtgttgtgcggcagcggcctgctgggcgtagcgagcggccatggcagcatggaggaccccatcagtcgcgtctacaactgctacctggagaatcccgagagtcccacgtcggcagcttgccaagcggcggtggcgctgagtggggcccaagcgttctatgattggaatgaggtgaacctggccgacgccgctggccggcatcgcgagctcattccggatggccaactgtgcagcgccgggcgggagaagtatcagggcctcgacctggcacgctccgactggacagccacttccttgtcctccggcgtctccttcacatacctctacaaggccaccgccccgcacttgggcttcttcgagttctacgtcaccaaggatggttacgagcccactgagccgctcaaatgggcagacttggaggactcgcccctcatcaacgtcaccgaccccacgcttgtcagcggctcctaccaaatccccggcaccacgccttccggcaagtccggccgccacctcatctacgtcatttggcagcgctccgacagccccgaggccttctactcctgctccgacgtcgacttcgacgtcgatgccctctctctccactccaccacc

SEQ ID NO: 115 - DNA, 705 bp, Onoclea sensibilis
atggggaggtcatggggagtggtgcaggctataattatggtgttgtgcggcagcggcctgctgggcgtagcgagcggccatggcagcatggaggaccccatcagtcgcgtctacaactgctacctggagaatcccgagagtcccacgtcggcagcttgccaagcggcggtggcgctgagtggggcccaagcgttctatgattggaatgaggtgaacctggccgacgccgctggccggcatcgcgagctcattccggatggccaactgtgcagcgccgggcgggagaagtatcagggcctcgacctggcacgctccgactggacagccacttccttgtcctccggcgtctccttcacatacctctacaaggccaccgccccgcacttgggcttcttcgagttctacgtcaccaaggatggttacgagcccactgagccgctcaaatgggcagacttggaggactcgcccttcatcaacgtcaccgaccccacgcttgtcagcggctcctaccaaatccccggcaccacgccttccggcaagtccggccgccacctcatctacgtcatttggcagcgctccgacagccccgaggccttctactcctgctccgacgtcgacttcgacgtcgatgccctctctctccactccacacctaatctagacttgtcatcttctggattggccaacttaattaatgtatgtgta

SEQ ID NO: 116 - DNA, 688 bp, Onoclea sensibilis
atggggaggtcatggggagtggtgcaggctataattatggtgttgtgcggcagcggcctgctgggcgtagcgagcggccatggcagcatggaggaccccatcagtcgcgtctacaactgctacctggagaatcccgagagtcccacgtcggcagcttgccaagcggcggtggcgctgagtggggcccaagcgttctatgattggaatgaggtgaacctggccgacgccgctggccggcatcgcgagctcattccggatggccaactgtgcagcgccgggcgggagaagtatcagggcctcgacctggcacgctccgactggacagccacttccttgtcctccggcgtctccttcacatacctctacaaggccaccgccccgcacttgggcttcttcgagttctacgtcaccaaggatggttacgagcccactgagccgctcaaatgggcagacttggaggactcgcccttcatcaacgtcaccgaccccacgcttgtcagcggctcctaccaaatccccggcaccacgccttccggcaagtccggccgccacctcatctacgtcatttggcagcgctccgacagccccgaggccttctactcctgctccgacgtcgacttcgacgtcgatgccctctctctccactccacacctaatctagacttgtccattctggattggccaactt

SEQ ID NO: 117 - DNA, 645 bp, Polystichum tripteron
atgggcaggtcatggggagttgtggctattatggtgttgtgcgccagcggcctgctgggcgtagcgagcggccatggcaccatgaacgaccccatcagtcgcgtctacgcctgcaggcaggagaatccggagcgacccactacgccggcttgcatagcggcggtggcgctgagtggggcccaagcgttctatgattggaatgaggtgaacctgccctttgtcaatggccggcaccgccagttcattccggatgggaaactctgcagcgccgggcggaacaagtataggggtctcgacctggcacgctccgactggacagccacaaacttgtcctccggcgtcgcctacacattcctctacagggtcaccgcccagcacaggggcttcttcgagttctacgtcaccgtggatggttacgaccccactgagccgctcaaatgggcagacttggaggaaacgccgttcatcaacgtcaccgaccccacagttgtaggcctcaactatgtaatccccggtaccacgcctgccagcaagaccggccgccacctcatctacgtcatttggcagcgctccgacagccccgaggccttctactcctgctccgacgtcaactttcccgatgccctgtctctccactccgccacc

SEQ ID NO: 118 - DNA, 645 bp, Polystichum tripteron
atgggcaggtcatggggagttgtggctattatggtgttgtgcgccagcggcctgctgggcgtagcgagcggccatggcaccatgaacgaccccatcagtcgcgtctacgcctgcaggcaggagaatccggagcgacccactacgccggcttgcatagcggcggtggcgctgagtggggcccaagcgttctatgattggaatgaggtgaacctgccctttgtcaatggccggcaccgccagttcattccggatgggaaactctgcagcgccgggcggaacaagtataggggtctcgacctggcacgctccgactggacagccacaaacttgtcctccggcgtcgcctacacattcctctacagggtcaccgcccagcacaggggcttcttcgagttctacgtcaccgtggatggttacgaccccactgagccgctcaaatgggcagacttggaggaaacgccgttcatcaacgtcaccgaccccacagttgtaggcctcaactatgtaatctccggcaccacgcctgccagcaagaccggccgccacctcatctacgtcatttggcagcgtaccgacagccccgaggccttctactcctgctccgacgtcaactttcccgatgccctgtctctccactccgccacc

SEQ ID NO: 119 - DNA, 645 bp, Polystichum tripteron
atgggcaggtcatggggagttgtggctattatgatgttgtgcgccagcggcctgctgggcgtagcgagcggccatggcaccatgaacgaccccatcagtcgcgtctacgcctgcaggcaggagaatccggagcgacccactacgccggcttgcatagcggcggtggcgctgagtggggcccaagcgttctatgattggaatgaggtgaacctgccctttgtcaatggccggcaccgccagttcattccggatgggaaactctgcagcgccgggcggaacaagtataggggtctcgacctggcacgctccgactggacagccacaaacttgtcctccggcgtcgcctacacattcctctacagggtcaccgcccagcacaggggcttcttcgagttctacgtcaccgtggatggttacgaccccactgagccgctcaaatgggcagacttggaggaaacgccgttcatcaacgtcaccgaccccacagttgtaggcctcaactatgtaatccccggtaccacgcctgccagcaagaccggccgccacctcatctacgtcatttggcagcgctccgacagccccgaggccttctactcctgctccgacgtcaactttcccgatgccctgtctctccactccgccacc

SEQ ID NO: 120 - DNA, 645 bp, Polystichum tripteron
atgggcaggtcatggggagttgtggctattatggtgttgtgcgccagcggcctgctgggcgtagcgagcggccatggcaccatgaacgaccccatcagtcgcgtctacgcctgcaggcaggagaatccggagcgacccactacgccggcttgcatagcggcggtggcgctgagtggggcccaagcgttctatgattggaatgaggtgaacctgccctttgtcaatggccggcaccgccagttcattccggatgggaaactctgcagcgccgggcggaacaagtataggggtctcgacctggcacgctccgactggacagccacaaacttgtcctccggcgtcgcctacacattcctctacagggtcaccgcccagcacaggggcttcttcgagttctacgtcaccgtggatggttacgaccccactgagccgctcaaatgggcagacttggaggaaacgccgttcatcaacgtcgccaaccccacagttgtaggcctcaactatgtaatctccggcaccacgcctgccagcaagaccggccgccacctcatctacgtcatttggcagcgtaccgacagccccgaggccttctactcctgctccgacgtcaacttcgtcgatgccctgtctctccactccgccacc

SEQ ID NO: 121 - DNA, 651 bp, Tectaria milnei
atggggaggtcatggggagtggtggctgttatggtggtgtgcgcaagcggcctattgagcgtagtgaggggccatggaagcatggaggaccccatcagtcgtgtgtatgcatgcttcctagagaatccggagcgtcccatatcagcagcttgccaggcggcagtggcaatgggtgggacgcaagccttctatgattggaatgcggtaagcctgccctatgctgctgggcggcaccgtgaactcatcccggatggccaattgtgcagtgctgggcgggccaagtatcggggcctggacctgcctcgtgacgattggccaggcacctccaatatgacctccggcgtcgccttcacatacaggtacaaggccaccgccccacacttgggctccttccagttctatgtcactcgggatggctacgatcccaccgagccgctcaaatgggcagacttggaggactcgcctttcatgaacgccaccagcacgcttgccccggactcctacctaatgtccggcaccacccctagcggcaaggctggccaccacctcatctacgccatttggcagcgcagcgacagccctgaggccttctactcctgctccgatgtcaccttcgacgtcgctgctgtctctgatctccactccaccacc

SEQ ID NO: 122 - DNA, 651 bp, Tectaria milnei
atggggaggtcatggggagtggtggctgttatggtggtgtgcgcaagcggcctattgagcgtagtgaggggccatggaagcatggaggaccccatcagtcgtgtgtatgcatgcttcctagagaatccggagcgtcccatatcagcagcttgccaggcggcagtggcaatgggtgggacgcaagccttctatgattggaatgcggtaagcctgccctatgctgctgggcggcaccgtgaactcatcccggatggccaattgtgcagtgctgggcgggccaagtatcggggcctggacctgcctcgtgacgattggccaggcacctccaatatgacctccggcgtcgccttcacatacaggtacaaggccaccgccccacacttgggctccttccagttccatgtcactcgggatggctacgatcccaccgagccgctcaaatgggcagacttggaggactcgcctttcatgaacgccaccagcacgcttgccccggactcctacctaatgtccggcaccacccctagcggcaaggctggccaccacctcatctacgccatttggcagcgcagcgacagccctgaggccttctactcctgctccgatgtcaccttcgacgtcgctgctgtctctgatctccactccaccacc

SEQ ID NO: 123 - DNA, 651 bp, Tectaria milnei
atggggaggtcatggggagtggtggctgttatggtggtgtgcgcaagcggcctattgagcgtagtgaggggccatggaagcatggaggaccccatcagtcgtgtgtatgcatgcttcctagagaatccggagcgtcccatatcagcagcttgccaggcggcagtggcaatgggtgggacgcaagccttctatgattggaatgcggtaagcctgccctatgctgctgggcggcaccgtgaactcatcccggatggccaattgtgcagtgctgggcgggccaagtatcggggcctggacctgcctcgtgacgattggccaggcacctccaatatgacctccggcgtcgccttcacatacaggtacaaggccaccgccccacacttgggctccttccagttctatgtcactcgggatggctacgatcccaccgagccgctcaaatgggcagacttggaggactcgcctctcatgaacgccaccagcacgcttgccccggactcctacctaatgtccggcaccacccctagcggcaaggctggccaccacctcatctacgccatttggcagcgcagcgacagccctgaggccttctactcctgctccgatgtcaccttcgacgtcgctgctgtctctgatctccactccaccacc

SEQ ID NO: 124 - protein, 215 aa, Polystichum tripteron
MGRSWGVVAIMVLCASGLLGVASGHGTMNDPISRVYACRQENPERPTTPACIAAVALSGAQAFYDWNEVNLPFVNGRHRQFIPDGKLCSAGRNKYRGLDLARSDWTATNLSSGVAYTFLYRVTAQHRGFFEFYVTVDGYDPTEPLKWADLEETPFINVTDPTVVGLNYVIPGTTPASKTGRHLIYVIWQRSDSPEAFYSCSDVNFPDALSLHSTT

SEQ ID NO: 125 - protein, 212 aa, Polystichum tripteron
MGRSWGVVAIMVLCASGLLGVASGHGTMNDPISRVYACRQENPERPTTPACIAAVALSGAQAFYDWNEVNIPNAPGRHRELISDGYLCSANRTKYAGLDLARSDWTATNLSSGVAYTFLYRVTAQHRGFFEFYVTVDGYDPTEPLKWADLEETPFINVTDPTVVGLNYVIPGTTPASKTGRHLIYVIWQRSDSPEAFYSCSDVNFPDALSLH

SEQ ID NO: 126 - protein, 214 aa, Davallia fejeensis
MGRSWGVVAIMVVCIMSGLVGIVSGHGSMEDPISRVYRCYLENPERPVSAACQAAVAMSGTQAFYDWNEVNIPNAAGRHRELISDGQLCSANRTKYAGLDLARADWLGTPLSSGVSFTFAYKATAPHLGFFEFYVTRDGYEPTEPLKWADLEDSPFINVTDPTLENGAYQISGTTPSGKSGRHLMYVIWQRSDSPEAFYSCSDVDFDVDALSLH

SEQ ID NO: 127 - protein, 212 aa, Didymochlaena truncatula
MGRSWGVVAIMVLCASGLLGVASGHGSMEDPISRVYACYLENPERPTSAACQAAVAVSGTQAFYDWNEVNQPFAAGRHRELIPDGELCSGGREKYKGLDLARADWPATSLPSGVNYTYLYKATAPHLGFFEFYITRDGYEPTEPLKWADLEDLPFINITNPTLVSGSYQIPGTTHASKTGRHLLYVIWQRSDSFEAFYSCSDVDFVNALSLH

SEQ ID NO: 128 - protein, 212 aa, Didymochlaena truncatula
MGRSWGVVAIMVLCASGLLGVASGHGSMEDPISRVYACYLENPERPTSAACQAAVAVSGTQAFYDWNEVNQPFAAGRHRELIPDGELCSGGREKYKGLDLARADWPATSLPSGVNYTYLYKATAPHLGFFEFYITRDGYEPTEPLKWADLEDLPFINITNPTLVSGSYQIPGTTPASKTGRHLLYVIWQRSDSFEAFYSCSDVDFVNALSLH

SEQ ID NO: 129 - protein, 212 aa, Humata tyermanii
MGRSWGVVAIMVMYIGGLLSIASGHGSMEDPISRVYRCYLENPESPTSAACQAAVAVSGAQAFYDWNEVNIADANGRHRELISDGQLCSANRSKYAGLDLARADWLGTTLSSGASFTFAYKATAPHLGFFEFYVTRDGYEPTDPLKWADLEDSPFINVTNPTLDNGAYQISGTTPAGKSGRHLIYVIWQRSDSPEAFYSCSDVDFVDALSLH

SEQ ID NO: 130 - protein, 215 aa, Cyrtomium fortunei
MGRSWGVVAIMVLCTSGLLGVASGHGTMGDPISRVYNCFQENPERPTSAACIAAVALSGTQAFYDWNEVNLPDVNGRHREFIPDGQLCSAGRDKYKGLDLARSDWTATNLSSGVAYTFLYRVTAQHRGFFEFYVTVDDYDPTVALKWEDLEETPFLNVTDPTVVGVNYQISGTTPASKTGRHLIYVIWQRSDSPEAFYACSDVDFVDAVSLHSTT

SEQ ID NO: 131 - protein, 229 aa, Adiantum hispidulum
MKKSWGVAVVVGVVALCLLGMASGHGSMQDPISRVYNCYLEGPERPTSAACIAAVAMSGTQPFYDWNEVNLPDAAGRHRELIPDGKLCSAGRDKYQGLDLARDDWVASLSSGVAYTFLYRVTAQHLGFFEIYVTRDTYDPTQALTWDDLEDSPFINVTNPSVVSTTLGNAYAIPTPTPSGKTGRHLIYVIWQRSDSPEAFYSCSDVEFDVASTVEDDVIISLRSAALDV

SEQ ID NO: 132 - protein, 215 aa, Polystichum acrostichoides
MGRSWGVVAIMVLCASGLLGVASGHGSMNDPISRVYNCRLENPESPTSAACIAAVALSGTQAFYDWNEVNLPDVNGRHRQLIPDGKLCSAGRDKYKGLDLARSDWVATNLSSGVAFTFLYRVTAQHRGFFEFYVTVDDYDPTELLKWEDLEETPFMNVTDPTVVGVNYEIPGTTPANKTGRHLIYVIWQRSDSPEAFYSCSDVDFVDAVSLHSTT

SEQ ID NO: 133 - protein, 217 aa, Thelypteris kunthii
MERAAWGVVGIIMVLCASGLLGVASGHGSMEDPISRVYLCYLENPERPTSAACQAAVALSGTQAFYDWNEVNIADAAGRHRELIPDGQLCSAGRDKYKGLDLARSDWVATNLSSGVAFTFLYRVTAEHRGFFEFYVTVDDYDPTELLKWEDLEATPFMNVTDPTVVGDNYEIPGTTPANKTGRHLIYVIWQRSDSPEAFYSCSDVVFADAVSLHSTT

SEQ ID NO: 134 - protein, 222 aa, Cyrtomium fortune (clivicola)
MGTLGRSWGAVAIMVLCASGLLGVASGHGSMNDPISRVYNCYLENPERPTSAACIAAVALSGTQAFYDWNEVNLPDANGRHRQLIPDGQLCSAGRDKYKGLDLARSDWTATNLSSGVAFTFLYRVTAQHRGFFEFYVTVDDYDPTVALKWEDLEETPFLNVTDPTVVGVNYQISGTTPASKTGRHLIYVIWQRSDSPEAFYACSDVDFVDAVSLHSTTLTLI

SEQ ID NO: 135 - protein, 215 aa, Polystichum tripteron
MGRSWGVVAIMVLFSSGLLGVASGHGSMGDPISRVYNCRQENPERPTTPACIAAVALSGAQAFYDWNEVNLPFVNGRHRQFIPDGKLCSAGRNKYRGLDLARSDWTATNLSSGVAYTFLYRVTAQHRGFFEFYVTVDGYDPTEPLKWADLEETPFINVTDPTVEGLNYVRVLRHRGCKSGRHLIYVIWQRSDSPEAFYSCSDVNFPDALSLHSAT

SEQ ID NO: 136 - protein, 215 aa, Didymochlaena truncatula
MGRSWGVVAIMVLCASGLLGVASGHGSMEDPISRVYACYLENPERPTSAACQAAVAVSGTQAFYDWNEVNQPFAAGRHRELIPDGELCSGGREKYKGLDLARADWPATSLPSGVNYTYLYKATAPHLGFFEFYITRDGYEPTEPLKWADLEDLPFINITNPTLVSGSYQIPGTTPASKTGRHLLYVIWQRSDSFEAFYSCSDVDFVNALSLHSTT

SEQ ID NO: 137 - protein, 229 aa, Asplenium antiquum
MRMGRSASCIRANMAIMLVLFWASCSCLLGIVSGHGSMEDPISRVYACFLENPERPTSAACIAAVALSGTQAFYDWNEVNQPNAAGRHREIIPDGQLCGAGRDKYKGLNLARADWPATTLSSDISFTYLFKATAPHRGFFEFYVTRDGYDPTEPLKWADLEDPPFLNVTDPTLASGSYQIPGTTPAGKTGRHLIYVIWQRSDSPEAFYSCSDVDFDSSDTVISLRSATT

SEQ ID NO: 138 - protein, 215 aa, Cyrtomium falcatum (Butterfieldii)
MGRSWGVVAIMVLCATGLLGVASGHGSMGDPISRVYNCFLENPERPTSAACIAAVALSGTQAFYDWNEVNLPDVNGRHRQFIPDGQLCSAGRDKYKGLDLARSDWTATNLSSGIAYTFLYRVTAQHRGFFEFYVTVDDYDPTVALKWEDLEETPFLNVTDPTVVGVNYQINGTTPASKTGRHLIYVIWQRSDSPEAFYACSDVDFVDAVSLHSTT

SEQ ID NO: 139 - protein, 218 aa, Onoclea sensibilis
MGRSWGVVQAIIMVLCGSGLLGVASGHGSMEDPISRVYNCYLENPESPTSAACQAAVALSGAQAFYDWNEVNLADAAGRHRELIPDGQLCSAGREKYQGLDLARSDWTATSLSSGVSFTYLYKATAPHLGFFEFYVTKDGYEPTEPLKWADLEDSPFINVTDPTLVSGSYQIPGTTPSGKSGRHLIYVIWQRSDSPEAFYSCSDVDFDVDALSLHSTT

SEQ ID NO: 140 - protein, 216 aa, Platycerium superbum
MRRSWVAVAVTLVVCAGSLLGVASGHGSMEDPISRVYGCYLENPENPTSAACIAAVAASGTQAFYDWNEVNQPFAAGQHRQIIPDGQLCSAGRDKYKGLDLARADWPATSLSSGVDYTFLFKATAPHRGYFEFYVTRDSYDPTEPLAWADLEDTPFINVTDPTLVSGSYQISSTTPSGKTGRHLIYVIWQRTDSTEAFYSCSDVDFDETLRLHSAT

SEQ ID NO: 141 - protein, 215 aa, Davallia tyermannii
MGRSWGVVAIMVMYIGGLLSIASGHGSMEDPISRVYRCYLENPESPTSAACQAAVAVSGAQAFYDWNEVNIADANGRHRELISDGHLCSANRTKYAGLDLACPDWLGTLLFSGVSYTFSYKATAPHLGFFEFYVTRDGYEPTDPLKWADLEDSPFINVTNPTLDNGAYQISGTTPAGKSGRHLIYVIWQRSDSPEAFYSCSDVDFVDALSLHSTT

SEQ ID NO: 142 - protein, 217 aa, Tectaria milnei
MGRSWGVVAVMVVCASGLLSVVRGHGSMEDPISRVYACFLENPERPISAACQAAVAMGGTQAFYDWNAVSLPYAAGQHRELIPDGQLCSAGRAKYRGLDLPRDDWPGTSNMTSGVAFTYRYKATAPHLGSFQFYVTRDGYDPTEPLKWADLEDSPFMNATSTLAPDSYLMSGTTPSGKAGHHLIYAIWQRSDSPEAFYSCSDVTFDVAAVSDLHSTT

SEQ ID NO: 143 - protein, 216 aa, Polystichium tsus-simense
MGRSWWGVLAVMVLCASGLLGVASGHGTMNDPISRVYNCFLENPESPTSAACIAAVALSGTQAFYDWNEVNLANAAGRHRELIPDGQLCSAGRDKYKGLDLARSDWTATNLSSGVAFTFLYRVTAQHRGFFEFYVTVDDYDPTELLKWEDLEETPFLNVTDPTVVGVNYEISGTTPASKTGRHLIYVIWQRSDSPEAFYSCSDVDFVDSLSLHSTT

SEQ ID NO: 144 - protein, 216 aa, Nephrolepis falcata
MGRSWWGAVAIVLAVCASGLLSVVSGQGSMAYPISRVYGCFLENPLSPTSAACNAAVALSGTQAFYDWNEVSLANASGQHRQLIPDGQLCSAGQAKYRGLDLARDDWPGTSLTSGVAYTFYYYATTLHLGFFEFYVTRDGYDATQPLKWADLEDSPFLNVTSTLAASSFQWSSITPSDKSGRHLIYVIWQRTDSPEAFYSCSDVDFDYAVSLHSTT

SEQ ID NO: 145 - protein, 213 aa, Nephrolepis exaltata (compacta)
MGRSWGVAAIVVAVCASGLLSVVSGHGSMQDPISRVYACYLENPERPTSAACQAAVALSGTQAFYDWNEVNLPNAAGRHRELIPDGQLCSAGRAKYQGLDQARNDWPHTDLISGVAFTFNYRATAPHLGIFEFYVTRDGYDATQPLKWADLEDSPFLTATSTLAPSSYQWPGTTPSGKSGRHLIYVIWQRTDSPEAFYSCSDVEFVDAVSLHS

SEQ ID NO: 146 - protein, 215 aa, Nephrolepis exaltata (Tiger Fern)
MGRSWGVAAIVVAVCASGLLSVVSGHGSMQDPISRVYACYLENPERPTSAACQAAVALSGTQAFYDWNEVNLPNAAGRHRELIPDGQLCSAGRAKYQGLDQARNDWPHTDLISGVAFTFNYRATAPHLGIFEFYVTRDGYDATQPLKWADLEDSPFLTATSTLAPSSYQWPGTTPSGKSGRHLIYVIWQRTDSPEAFYSCSDVEFVDAVSLHSTT

SEQ ID NO: 147 - protein, 215 aa, Humata termanii
MGRSWGVVAIMVMYIGGLLSIASGHGSMEDPISRVYRCYLENPESPTSAACQAAVAVSGAQAFYDWNEVNIADANGRHRELISDGQLCSANRSKYAGLDLARADWLGTTLSSGASFTFAYKATAPHLGFFEFYVTRDGYEPTDPLKWADLEDSPFINVTNPTLDNGAYQISGTTPAGKSGRHLIYVIWQRSDSPEAFYSCSDVDFVDALSLHSTT

SEQ ID NO: 148 - protein, 220 aa, Adiantum tenerum (Scutum Roseum)
MGWCRSWGVVAVMVLCTSGLLGVASGHGSMKDPISRVYNCYLENPERPTSAACQAAVALSGTQAFYDWNEVNLPNAAGRHRELIPDGELCSAGREKYQGLDLARADWTATSLTSGLDSFTWLYKATAPHLGFFEFYVTRDGYDPTEALTWADLEDSPFINVTNPALVSGDYQISGTIPAGKSGRHLIYVIWQRSDSPEAFYSCSDVDFVDDALISLRSAT

SEQ ID NO: 149 - protein, 215 aa, Polystichum setiferum (compacta)
MGRSWGVAAIMVLCASGLLGVASGHGTMHDPISRVYNCFLENPESPTSAACIEAVEVSGTQPFYDWNEVNLANAAGRHRELIPDGKLCSAGRDKYKGLDLARSDWVATNLSSGVAFTFLYRVTAEHRGFFEFYVTVDDYDPTELLKWEDLEETPFMNVTDPTVVGANYEIPGTTPANKTGRHLIYVIWQRSDSPEAFYSCSDVVFADAVSLHSTT

SEQ ID NO: 150 - protein, 215 aa, Polystichum setiferum (compacta)
MGRSWGVAAIMVLCASGLLGVASGHGTMHDPISRVYNCFLENPESPTSAACIEAVEVSGTQPFYDWNEVNLPDVNGRHRELIPDGKLCSAGREKYKGLDLARSDWVATNLSSGVAFTFLYRVTAEHRGFFEFYVTVDDYDPTELLKWEDLEATPFMNVTDPTVVGDNYEIPGTTPANKTGRHLIYVIWQRSDSPEAFYSCSDVVFADAVSLHSTT

SEQ ID NO: 151 - protein, 215 aa, Lepisorus bicolor
MRSWGVVAIMVAVCASGLLGVASGHGSMSDPISRVYRCRLENPERPTSAACIAAVALSGKQAFYDWNEVNLPFANGRHRELIPDGKLCSAGRDKYKGLDLPRADWLATSLSSGSAYTFLYRATAPHLGYFEFYVTRDSYDPTQPLAWSDLEDSPFIKVTNPPLVSGFYEFPGTTPSGKTGRHLIYVIWQRTDSTEAFYSCSDVDFDEALSLSSTI

SEQ ID NO: 152 - protein, 217 aa, Pyrrosia lingua (Ogon)
MRTRVWGVVAFMVAVCACDLLGLASGHGSMGDPVSRVLNCYLENPERPTSAACIAAVALSGTQAFYDWNEVNLASACGRHRELISDGELCSAGRDKYKGLNLARADWVATSLSSGVDYTFLFNATAAHLGYFEFWVTRDSYDPTQPLAWADLEDSPFINITNPTIVSDAYQVPATTPSGKTGRHLIYVIWQRTDSTEAFYSCSDVDFDEALPLSSTT

SEQ ID NO: 153 - protein, 224 aa, Blechnum appendiculatum
MKKSSGVVVVVVAAILLLCLLGVANGHGSMQDPISRVYNCFLENPESPTSAACQAAVAVAGTQPFYDWNEVNLANANGRHRELISDGMLCSANRSKYHGLDLARADWTATSLSSGVAYTFLYRVTAHHRGFFEFYITRDSYDPTQPLAWADLEDSPFINITDPTTVSTTLGEAYEISGTTPASKSGRHLIYVIWQRSDSPEAFYSCSDVDFSADALISLRSAVL

SEQ ID NO: 154 - protein, 215 aa, Polystichum munitum
MGRSWGVVAIMVLCASGLLGVASGHGTMNNPISRVYNCRLENPERPTSAACIAAVALSGTQAFYDWNEVNLPDVNGRHRELIPDGKLCSAGRDKYKGLDLARSDWVATNLSSGVAFTFLYRVTAQHRGFFEFYVTVDDYDPTELLKWEDLEETPFMNVTDPTVVGVNYEIPGTTPANKTGRHLIYVIWQRSDSPEAFYSCSDVDFVDAVSLHSTT

SEQ ID NO: 155 - protein, 217 aa, Stenochiaena tenuifolia
MGMGRSNSSKVVAIVVLCSGLLSLVSGHGSMQNPISRVLNCYLENPERPTSAACQAAVAMSGTQAFYDWNEVNLPNAAGRHRQLIPDGQLCSAGRQKYRGLDLARDDWEATTLSSGTAFTYNYRATAPHLGFFEFYVTRDGYEPTEPLKWSDLQDSPFINVTTTLSSDSYQITGTTPAGKSGRHLIYVIWQRSDSPEAFYSCSDVEFDVALSLHSAT

SEQ ID NO: 156 - protein, 231 aa, Asplenium bulbiferum (G.Forst.)
MRMGRSTSCMGANMAFMLLLLLFWASCCCLLGKVSGHGSMEDPISRVYACFLENPERPTSAACQAAVALSGTQAFYDWNEVNQPNAAGRHREIIPDGQLCSGGREKYQGLDLARDDWTATSLSPNVSFTFLYKATAPHRGFFEFYVTRDGYDPTEALTWADLEEPPFINVTDPTVASGAYQIPGTTPAGKTGRHLIYVIWQRSDSPEAFYSCSDVDFESADTVNISLRSTT

SEQ ID NO: 157 - protein, 221 aa, Athyrium filix-femina
MGRSWGVVAILMVLCGCLLGVASGHGSMEDPISRVYNCYLENPESPTSAACQAAVALGGPQPFYDWNEVNQPNADGHSREIIPDGQLCSGGREKYKGLDLARSDWTATSLSSGVAFTFLFKATAPHAGFFEFYVTQDGYDPTEPLKWADLEDSPFINVTDPTLLSGSYQIPGTTPAGKSGRHLIYVIWQRSDSPEAFYSCSDVDFVDALSSDLHSTMAPIA

SEQ ID NO: 158 - protein, 231 aa, Adiantum capillus-veneris
MGMKMSWEVALAEIVALCLLGMASSHGTMQDPISRVYNCFLENPERPTSAACQAAVALGGTQPLYDWNEVNIHDAAGNHRDLIPDGKLCSAGRQKFQGLDLARADWIATSLSSGVDVDYTFLYRATAPHLGFFEFYITRDTYDPTQPLAWGDLEDSPFINITNPSIVSTTLGPAYSIPSTTPFSKSGRHLIYVIWQRTDSLEAFYSCSDVDFSTSSIEDDVIVSLRSAALL

SEQ ID NO: 159 - protein, 231 aa, Asplenium nidus var plicatum
MRMGRSISRMAARMAIMLVLCWAISCCLLGTVSGHGSSEDPMSRVYGCYLQNPERPASAACRAAVAMSGTQAFYDWNEVNQPHAAGRHREIIPDGQLCGGGRAKYRGLNLARADWWSTPLYSNTPFMFLYRATAPHRGFFEFYVTRDGYDPTEPLKWSDLEYPPFINVTDPTLAFGAYKIPGFTPYGKTGRHLIYIIWQRSDSPEAFYSCSDVDFVDFKSDETVIPLHSTT

SEQ ID NO: 160 - protein, 215 aa, Polystichum polyblepharum
MGRSWGVVAIMVLCASGLLDVASGHGSMNDPISRVYNCRLENPESPTSDACIAAVALSGTQAFYDWNEVNLPNAAGRHRELIPDGKLCSAGRDKYKGLDLARSDWVATNLSSGVAFTFLYRVTAQHRGFFEFYVTVDDYDPTELLKWEDLEETPFMNVTDPTVVGVNYEMAGTTPANKTGRHLIYVIWQRSDSPEAFYSCSDVDFVDAVSLHSST

SEQ ID NO: 161 - protein, 215 aa, Adiantum venustum
MGRSWGDVVAIMVLCASGLLGVASGHGSMQDPISRVYNCYLEGPESPTSAACIAAVALSGTQAFYDWNEVNQPNAAGRHREIIPDGQLCSGGRDKYSGLDLARSDWTATSLSSNVSYTYLFKATAPHKGFFEFYVTRDSYEPTEALKWADLEDSPFINITDPTLDSGAYQIPGTTPAGKSGRHLIYVIWQRSDSGEAFYACCDVDFDVDVLHSTT

SEQ ID NO: 162 - protein, 233 aa, Actiniopteris australis
MRQGSSIADMSVRMGGVNAVAIILLLCCASSGLLGIARGHGSMQDPISRVYACYLENPERPTSAACQAAVALSGTQAFYDWNEVNQPFAAGRHREIIPDGQLCSGGRTKYAGLDLARDDWTATSLSAGISYTFLYRGTAPHLGFFEFYVTRDGYDPTEPLKWADLEDPPFINITNPTLVSGVYQIPGTTPAGKTGRHLIYVIWQRTDSPEAFYSCSDVVFSDDAALYLRSTTE

SEQ ID NO: 163 - protein, 231 aa, Marsilea crenata
MRRSGMSSSVLAAVAAGVLLVAALGSHVAYGHGSMKEPISRAYNCYLEIADNATSDACGAAAALCIPEAFNDWNAVLIPDVAGRHRQLIPDGQLCSAGRAKYAGLNLASVDWEAATLAAGVNYTFLYKAVVVHKGYFEFYVTKDGYDATQALTWSDLEDAPFVNVTDPIVNSDSDFEIPGTIPSGKSGRHVIYVIWQRTDSPEAFYSCSDVDFDDTISDDTISDTVLHASS

SEQ ID NO: 164 - protein, 229 aa, Asplenium prolongatum x Asplenium antiquum (Kurata)
MRMGRSASCIRANMAIMLVLFWASCCCLLGIVSGHGSMEDPISRVYACYLENPERPTSAACIAAVALSGTQAFYDWNEVNQPNAAGRHREIIPDGQLCSGGREKYQGLDLARADWTATSLTSGITFTFLYKATAPHRGFFEFYVTRDTYDPTEPLTWADLEDTPFINATDPTLASGSYQIPGTTPAGKTGRHLIYVIWQRSDSPEAFYSCSDVDFESSDTVISLRSATT

SEQ ID NO: 165 - protein, 229 aa, Adiantum raddianum (Fritz Luthi)
MGMKMSWEVALAEIVALCLLGMASSHGTMQDPISRVYNCFLENPERPTSAACQAAVALGGTQPLYDWNEVNIHDAAGNHRDLIPDGKLCSAGRQKFQGLDLARADWIATSLSSGVDYTFLYRATAPHLGFFEFYITRDTYDPTQPLAWGDLEDSPFINITNPSIVSTTLGPAYSIPSTTPFSKSGRHLIYVIWQRTDSLEAFYSCSDVDFSTSSIEDDVIVSLRSAALL

SEQ ID NO: 166 - protein, 227 aa, Asplenium australasicum
MRMGRSTSRMAARMAITLLLCWASCCLLGTVSGHGSMLDPISRIYACFLENPERPTSAACQAAVALGGTQPLYDWNEVNQPNAAGRHREIIPDGQLCGGGREKYQGLNLARADWPATSLSSNTAFTFLYIATAPHRGFFEFYVTRDGYDPTELLKWADLEYPPFLNVTDPTLASGNYQIPGTTPAGKTGRHLIYVIWQRSDSPEAFYSCSDIDFESDETVISLHSTT

SEQ ID NO: 167 - protein, 227 aa, Asplenium australasicum
MRMGRSTSRMAARMAITLLLCWASCCLLGTVSGHGSMLDPISRIYACFLENPERPTSAACQAAVALGGTQPLYDWNEVNQPNAAGRHREIIPDGQLCSGGREKYKGFDLPRADWPATTLVSNISFTYLYKATAPHRGFFEFYVTRDGYDPTELLKWADLEYPPFLNVTDPTLASGNYQIPGTTPAGKTGRHLIYVIWQRSDSPEAFYSCSDIDFESDETVISLHSIT

SEQ ID NO: 168 - protein, 216 aa, Thelypteris palustris
MGRSWGVVGIMVLCLLGVASGHGTMQDPISRVYNCRLENPERPTSAACIAAVALSGTQAFYDWNEVNLANAAGRHRELIPDGQLCSAGRVKYQGLDLARSDWTATSLSSGVSFTFLYRVTAQHLGFFEFYVTQDGYDPTEPLKWADLEDSPFINVTNPTVVSTSLGPAYQIAGTTPAGKSGRHLIYVIWQRSDSPEAFYSCSDVDFVDALSLHSTA

SEQ ID NO: 169 - protein, 230 aa, Asplenium dimorphum x Asplenium difforme
MRMGRSTSCMGANMAIVLLLLLFWASCCCLLGKVSGHGSMEDPISRVYACFLENPERPTSAACQAAVALSGTQAFYDWNEVNLPNAAGRHREIIPDGQLCSGGREKYKGLDLARADWTATSLSPNVSFTFLYKGTAPHRGFFEFYVTRDGYDPTEALTWADLEEPPFINVTDPTLASGAYQIPGTTPAGKTGRHLIYVIWQRSDSPEAFYSCSDVDFESDDTVVSLRSTT

SEQ ID NO: 170 - protein, 215 aa, Matteuccia struthiopteris
MGRSWGVVAIMVLCASSLLGVVSGHGSMADPISRVYGCRLEGPESPTSAACQAAVALSGTQAFYDWNEVNQPFAAGRHRELIPDGQLCSGGRVKYQGLDLARSDWPATNLSSGVSFTFLYEVTATHLGYFEFYVTRDGYQPTEPLKWADLEDSPFLTATTTHESSSYIIPGTTPSAKSGRHLIYLIWQRTDSPEAFYSCSDVDFVDALSSLHSTN

SEQ ID NO: 171 - protein, 217 aa, Athyrium filix-femina (angustum)
MGRSWGVVAILMVLCGCLLGVASGHGSMEDPISRVYNCYLENPESPTSAACQAAVALGGTQPLYDWNEVNQPNAAGQSREIIPDGQLCSGGREKYQGLDLARSDWTATSLSSGVAFTFLFKATAPHLGFFEFYVTQDGYDPTEPLKWADLEDSPFINVTDPTLLSGSYQIPGTTPAGKSGRHLIYVIWQRSDSPEAFYSCSDVDFVDALSSDLHSTT

SEQ ID NO: 172 - protein, 228 aa, Adiantum pubescens (Bronze)
MKKSWGVTAVVGVIALCLLDVASGHGSMQDPISRVYNCFLENPERPTSAACIAAVAMSGTQPFYDWNEVNLADANGRHRELIPDGKLCSAGRDKYQGLDQARDDWVATSLSSGVAYTFLYRVTAPHLGFFEFYVTRDTYDPTQALAWDDLEDSPFINITNPSVVSTTLGNAYSIPGTTPSGKTGRHLIYVIWQRSDSREAFYSCSDVDFPASTVEDDVIISLRSAALV

SEQ ID NO: 173 - protein, 215 aa, Blechnum niponicum
MGRSWGVVAIMVLCASGLLGVASGHGSMDDPISRVYNCYLENPERPTSAACQAAVALSGTQAFYDWNEVNQPFAAGRHREIIPDGQLCSGGREKYQGLDLARSDWTATSLSSGVSFTYLYKATAPHLGFFEFYVTVDGYQPTEPLKWSDLEDPPFINVTNPTLVSGSYQIPGTTPAGKTGRHLIYVIWQRSDSPEAFYSCSDVDFADALSLHSTT

SEQ ID NO: 174 - protein, 215 aa, Platycerium wandae
MGKPWRVVVAIVVVCASGLLGVASGHGSMGEPISRVYNCYLENPERPTSAACIAAVALSGTQAFYDWNEVNLPFAAGRHRELIPDGQLCSAGRDKYKGLDLARADWVATSLSSGVSYTFLYRATAPHQGYFEFYVTKDSYDPTEPLAWADLEDTPFINITDPTLVSGSYQIPSTTPSDKTGRHLIYVIWQRTDSPEAFYSCSDIDFDDTLPLHST

SEQ ID NO: 175 - protein, 214 aa, Nephrolepis cordifolia (Duffii)
MGRSWRVVAIMVVCASGLLSVVRGHGSMEDPLSRVYGCFLENPESPTSAACQAAVAMSGTLAFYDWFDVSLPNASGRHRELIPDGQLCGAGLTKYQGLNLARDDWTATSLTSGVSFTYLYKAAARHLGFFEFYVTRDGYDPTEPLKWADLEDLPFMNVTSTLDEESYQIPGTTPSGKAGRHLIYVIWQRSDSPEAFYSCSDVDFVDAVSLHSTT

SEQ ID NO: 176 - protein, 224 aa, Adiantum raddianum (Fragrans)
MGMKMSWEVALAEIVALCLLGMASSHGTMQDPISRVYNCFLENPERPTSAACQAAVALGGTQPLYDWNEVNIHDAAGNHRDLIPDGKLCSAGRQKFQGLDLARADWIATSLSSGVDYTFLYRATAPHLGFFEFYITRDTYDPTQPLAWGDLEDSPFINITNPSIVSTTLGPAYSIPSTTPFSKSGRHLIYVIWQRSDSPEAFYACSDIDFSTSSDMISLRSAVL

SEQ ID NO: 177 - protein, 216 aa, Platycerium bifurcatum (Netherlands)
MGKPWRVVVAIVVVCASGLLGVASGHGSMGDPISRVYNCYLENPERPTSAACIAAVALSGTQAFYDWNEVNLPFAAGRHRELIPDGQLCSAGRDKYKGLDLARADWVATSLSSGVSYTFLYRVTAPHRGYFEFYVTKDSYDPTEPLAWADLEDTPFINITDPTIVSGSYQISSTTPSDKTGRHLIYVIWQRTDSPEAFYSCSDVDFDDTLPLHSST

SEQ ID NO: 178 - protein, 221 aa, Pyrrosia polydactyla
MRMGMRMRLWGVVAFMVAVCAGELLDQASGHGSMGDPVSRVLNCYLENPENPSSAACIAAVAASGTQAFYDWNEVNLAFAAGQHRTLIPDGELCSAGREKYKGLNLARADWVATSLSSGANYTFLYRATAPHLGYFEFYVTQDSYDPTEPLAWADLEDSPFINVTNPALVSGSYRIAGTTPSGKTGRHLIYVIWQRTDSPEAFYSCSDVDFDEAVSLSSTT

SEQ ID NO: 179 - protein, 222 aa, Blechnum brasiliense
MKKPWGVVVVVAILLLCLLGVASGHGSMQDPISRVYNCYLENPERPTSAACQAAVAMSGTQAFYDWNEVNLANASGRHRELIPDGKLCSAGRDKYRGLDLARADWTATSLSSGVAYTFLHRVTARHLGFFEFYITRDSYDPTELLTWADLEDSPFINITNPTTVSTSLGNAYQIPGTTPAGKSGRHLIYVIWQRSDSPEAFYSCCDVDFSSDTLISLRSAAL

SEQ ID NO: 180 - protein, 222 aa, Blechnum SP. (Silver Lady)
MKKPWGVVVVVAILLLCLLGVASGHGSMQDPISRVYNCYLENPERPTSAACQAAVAMSGTQAFYDWNEVNLANASGRHRELIPDGKLCSAGRDKYRGLDLARADWTATSLSSGVAYTFLHRVTARHLGFFEFYITRDSYDPTEPLTWADLEDSPFLNITDPTTVGTPLGDAYEIPGTTPDGKSGRHLIYVIWQRSDSPEAFYSCCDVDFSSDTLISLRSAAL

SEQ ID NO: 181 - protein, 223 aa, Pteris cretica (Mayi)
MGSRSVGGGGAGAIYCMLLICCVSSGLLGIASGHGTMLDPFSRVYACRFFENPERPTSPACQAAVAASGTQAFYDWNEVNQPFAAGRHREIIPDGQLCSGGRDKYKGLDLARNDWPATSLSSNIPFTYLYIASAPHRGFFEFYVTQDGYDPTQPLKWADLEYPPFINITDPTLLSGSYQIPGTTPAGKSGRHLIYVIWQRSDSPEAFYSCSDVDFVDSLHASV

SEQ ID NO: 182 - protein, 221 aa, Cystopteris fragilis
MGRVNLLAILVLCASCCAGLLGVASGHGTMEDPISRVYNCFLENPERPTSAACQAAVALSGTQAFYDWNEVNLADAAGRHRELIPDGQLCSAGREKYRGLDLARSDWVATSLSSGVSTTFLYKATAPHLGFFEFYVTRDGYDPTEALKWSDLEDSPFLNVTDPTLLSSPYVYQIPGTTPAGKSGRHLIYVIWQRSDSPEAFYSCSDVAFDDAQLVSLHSTT

SEQ ID NO: 183 - protein, 220 aa, Dryopteris filix-mas
MGRSWGVVQAIIMVLCGSGLLGVASGHGSMEDPISRVYNCYLENPESPTSAACQAAVALSGAQAFYDWNEVNLADAAGRHRELIPDGQLCSAGREKYQGLDLARSDWTATSLSSGVSFTYLYKATAPHLGFFEFYVTKDGYEPTEPLKWADLEDSPFINVTDPTLVSGSYQIPGTTPSGKSGRHLIYVIWQRSDSPEAFYSCSDVDFSSDALISLGSAVL

SEQ ID NO: 184 - protein, 219 aa, Bolbitis cladorrhizans
MGRSLGAVVITLVLCAGGLLSLASGHGSMEDPISRVYRCYLENPESPTSAACQAAVALSGTEAFSGYAWSAVLANAAGQHRQLIPDGQLCSAGQELYAGLDLPRADWPATSLSSGVAFTYLYKAAIPHMGFFEFYITRDGYEPTEPLKWADLEDSPFLNVTDPPLVSSSYQIPGSTPAGKSGRHLIYVIWQRSDSPQAFYSCSDVDFVDATLSQLHSTT

SEQ ID NO: 185 - protein, 220 aa, Dryopteris filix-mas
MKKSWGVVVVVVVALVLLCLLGTASGHGSMQDPISRVYNCYLENPENPTSAACKAVVAVGGTQPLYDWNEVNLANAAGRHRELIPDGRLCSAGRDKYRGLDLARDDWPATSLSSGVDYTFLYRATAPHLGFFEFYVTRDSYDPTQPLAWADLEDLPFINVTNPALNAGAYQIPGTMPAGKSGRHLIYVIWQRSDSPEAFYSCSDVDFSSDALISLRSAVL

SEQ ID NO: 186 - protein, 218 aa, Pyrrosia lanceolata
MRTRSWGVVAFMVAVCAGDLLGLASGHGSMGYPVSRVLNCFLENPESPTSAACTAAVAMSGTQAFYDWNEVNLPFANGQHRDLIPDGQLCSAGRAKYAGLDLARDDWEATFLSSATSYTLLYRVTARHLGYFEFYVTRDSYNSTQPLAWADLEDSPFINITNPTVDSGYYQVPVDTPSGKTGRHLIYVIWQHTDSLEAFYSCSDVEFDVEVPSLRSTT

SEQ ID NO: 187 - protein, 218 aa, Athyrium filix-femina
MGRSWGGVVAIMVLCGCLLGVASGHGSMEDPISRVYNCYLENPESPTSAACQAAVALSGTQAFYDWNEVNQPFAAGQSREIIPDGQLCSGGREKYKGLDLARSDWTATSLSSGVAFTFLFKATAPHAGFFEFYVTQDGYDPTEPLKWADLEDSPFINVTDPTLVSGSYQISGTTPAGKSGRHLIYVIWQRSDSPEAFYSCSDVEFVDDALSSDLHSTT

SEQ ID NO: 188 - protein, 218 aa, Colysis wrightii (Monstifera)
MGRAWVVVAIMVAVCASGLLSFASRTRGHGSMGDPISRVLRCREENPENPTSPACIAAVALSGKQAFYDWNEVNLPFADGQHQKLIPDGQLCGAGRDKYKGLNLARADWLATSLSAGAPYTFLFLASAPHLGYFEFYVTRDSYDPTQPLAWADLEDSPFLTTTTTLDSSSYIIPGTTPAGKTGRHLIYLIWQRTDSPEAFYSCSDVDFEEAISLSSTT

SEQ ID NO: 189 - protein, 219 aa, Coniogramme venusta
MGRSSSWEGVLVVVVCCASGLLGVASGHGSMGSPISRVYNCRQENPERPTSAACREAVRISGTQAFYDWNEVNLPVASGRHRELIPDGKLCSAGRTKYAGLDLARSDWVSTVLPSGVPYTFLYRVTARHVGFFEFYVTRDGYQPSEPLKWSDLEEPPFINVTNPTMSGGFYRIPGTTPPAKAGRHLIYVIWQRSDSPEAFYSCSDAVFGDALSLQYSST

SEQ ID NO: 190 - protein, 217 aa, Platycerium coronarium
MRRSWGVVAVIMLAVCAVGMLGVASGHGSMEDPISRVYRCFLENPERPTSAACIAAVALSGTQAFYDWNEVNLPFAAGRHRELIPDGQLCSAGRDKYKGLDLARDDWVATSLSSGVNYTFLYKATAPHRGYFEFYVTRDSYDPTEPLAWADLEDTPFINVTDPDLASGSYQISSTTPSGKTGRHLIYVIWQRTDSPEAFYSCSDILFDEAVALYSTA

SEQ ID NO: 191 - protein, 218 aa, Cystopteris bulbifera
MGRVNLMAILALCASFCAALLGVASGHGSMQDPISRVYNCFLENPERPTSAACQAAVALSGTQAFYDWNEVNLANADGRHRELIPDGQLCSAGREKYQGLDLARADWTATSLSSGISYTFLYKATAPHLGFFEFYVTRDGYDPTEALKWSDLEDSPFLNVTNPTLVSGSYQIPVTTPAAKSGRHLIYVIWQRSDSPEAFYSCSDVDFDDALVSLHSTT

SEQ ID NO: 192 - protein, 217 aa, Platycerium ridleyi
MRRSWGVMAVILLAVCACGLLGVASGHGSMEDPISRVYGCYLENPERPTSAACIAAVALSGTQAFYDWNEVNQPFAAGRHRELIPDGQLCSGGRDKYKGLDLARDDWEATSLSSGANYSFLFKATAPHRGYFEFYVTQDSYDPTEPLAWGDLESTPFINVTDPDLFSGSYQISSTTPPGKTGRHLIYVIWQRTDSPEAFYSCSDVLFDEAVALYSTA

SEQ ID NO: 193 - protein, 215 aa, Dryopteris marginalis
MGRSWGVVAIIMVLCGSGLLGVASGHGSMQDPISRVYNCYLENPERPTSAACQAAVALSGTQAFYDWNEVNQPFAAGRHREIIPDGQLCSAGREKYRGLDLARSDWVATSLSSGVNYTYLYKATAPHLGFFEFYVTQDGYNSSEPLKWADLEDSPFINVTTTLDSASYQIPGTTPAGKNGRHLIYVIWQRSDSPEAFYSCSDVDFADALSLHSTT

SEQ ID NO: 194 - protein, 216 aa, Microsorum musifolium (Blume)
MRRSWGVLAIVMAVCASGLFGVASGHGSMEHPISRVYQCYREGPENPKSPACIAAKGLSGAQAFYDWNEVNQPFADGRHQEIIHDGHLCSGGRDKYRGLDLPRADWVATSLSAGKPYTFLYRATAHHLGYFEFYVTRDGYDPTKPLAWADLEDSPFINVTNPTLVSGSYRIPHTTPASKTGRHLIYVIWQRTDSFEAFYSCSDVVFDEALSLSSTI

SEQ ID NO: 195 - protein, 216 aa, Elaphoglossum SP.
MRRSWEVVALIMVVCACGLLGVASGHGSMEDPISRVYRCYLEGVENPTSAACIAAIEVSGKQAFYDWNEVNQPLAAGRHREIIPDGELCSGGREKYKGLDLARADWLATSLSSGVDYTFLYKATAEHKGYFEFYVTQDSYDPTEPLKWSDLEDTPFINVTQPLLVSGSYQIPGTTPSGKTGRHLIYVIWQRTDSAEAFYSCSDVNFDDALPIYSAT

SEQ ID NO: 196 - protein, 214 aa, Dryopteris lepidopoda
MGRSWGVVAIMVLCGSGLLGVASGHGSMEDPISRVYNCYLENPERPTSAACQAAVALSGTQAFYDWNEVNQPFAAGRHREIIPDGQLCSGGREKYRGLDLARSDWEATSLSSGVSYTYLYKATAPHLGFFEFYVTQDGYNSSEPLEWADLEDSPFINVTTTLDSASYQIPGTTPAGKTGRHLIYVIWQRSDSPEAFYSCSDVDFVDALSLHSTT

SEQ ID NO: 197 - protein, 214 aa, Polystichum lepidocaulon
MGRSWGVVAIMVLFASASGLLGVANGHGSMGNPISRVYNCRLENPERPTSAACIAAVALSGTYDWSEVNLPNANGRHRELIPDGKLCSAGRDKYKGLDLARSDWTATNLSSGVAYTFLYRVTAEHRGFFEFYVTVDDYEPTELLKWEDLEETPFLNVSDPTVVGNNYEISGTTPASKTGRHLIYVIWQRSDSPEAFYSCSDVDFVDTLSLHSTT

SEQ ID NO: 198 - protein, 215 aa, Polystichum polyblepharum (C.)
MGRSWGVVAIMVLCASGLLGVASGHGTMNDPISRVYNCRLENPESPTSAACIAAVALSGTQAFYDWNEVNLPNAAGRHRELIPDGKLCSAGRDKYKGLDLARSDWVATNLSSGVAFTFLYRVTAQHRGFFEFYVTVDDYDPTELLKWEDLEETPFMNVTDPTVVGVNYEMAGTTPANKTGRHLIYVIWQRSDSPEAFYSCSDVDFVDAVSLHSST

SEQ ID NO: 199 - protein, 216 aa, Lecanopteris sinuosa
MMRSWGVAAIMMAVCASGLLGVASGHGSMADPISRVYRCRLENPERPTSPACIAAVALSGTQAFYDWNEVNLPFAAGRHRQLIPDGQLCSAGRNKYKGLDLARADWLATSLSPGANYTFLYRATAPHAGYFEFYVTRDSYDPTEQLAWADLEDSPFITITNPTLVNGYYQIPNTVPAGKTGRHLIYVIWQRTDSPEAFYSCSDVDFDDALRLHYST

SEQ ID NO: 200 - protein, 215 aa, Aglaomorpha splendens
MRRSWGVVVILVVCVCGLLGVASGHGSMGDPISRVYGCRLENPESPTSAACIAAVAVSGTQAFYDWNEVNQPNANGRHREIIPDGELCSAGRVKYAGLDLARDDWVATSLSSGVNYTFLFVATAPHLGYFEFYVTQDSYDPTQPLKWSDLEATPFINVTDPTLLNGSYQIPSSTPSGKTGRHLIYVIWQRTDSPEAFYSCSDVDFDVALPLYSST

SEQ ID NO: 201 - protein, 216 aa, Polypodium formosanum
MKRSWGVAAIVMALSTCGLIGVASGHGSMGDPISRVYRCYRENPERPTSPACIAAVALSGKQAFYDWNAVNLFNANGRHRELIPDGQLCSAGRAKYKGLDLPRADWLATSLSSGVNFTFLYRVTARHLGYFEFYVTRDGYDPSEPLAWADLEDSPFIKITNPSVVSNSYVIPGITPAGKTGRHLIYVIWQRTDSQEAFYSCSDIDFDEAVPLYSTT

SEQ ID NO: 202 - protein, 214 aa, Nephrolepis obliterata (Sunjest)
MGRSWGVVAIMVVCACGLLSVVRGHGSMEDPISRVYGCYLENPESPKSAACQAAVALSGTQAFYDWNEVNLPDVAGRHRAVIPDGQLCSAGRAKYQGLNLARADWPATSLTSGVSFTYLYKVTAKHLGFFEFYVTQDGYDPTEPLKWADLEDLPFMNVTSTFDDESYQMSGTTPSGKAGRHLIYVIWQRSDSPEAFYSCSDVDFVDAVSLRSTT

SEQ ID NO: 203 - protein, 215 aa, Deparia acrostichoides
MGRSWGVVAIMVLCASGLLGVASGHGSMEGPISRVLNCYLENPERPTSGACIAAVALGGTQPFYDWNEVNLADADGRHRELIPDGQLCSAGREKFKGLDLARSDWPATSLSSGVAFTYLYKATAPHAGFFEFYVTRDGYKPTEPLKWADLEEPPFINVTDPKLVSGSYQIPGTTPAGKAGRHLIYVIWQRSDSPEAFYSCSDVDFVEALSLHSTT

SEQ ID NO: 204 - protein, 216 aa, Aglaomorpha sp. (Roberts)
MRRSWPGVVAIMVVCACGLLGVASGHGSMQDPISRVYRCRLENPERPTSAACIAAVALSGTQAFYDWNEVNQPFANGRHREIIPDGQLCSAGRAKYRGLDLARADWLAPSLSSGVDYTFLYIATAPHLGYFEFYITRDSYDPTEPLKWSDLEDSPFINVTNPSLVSGSYQIPGTTPSNKTGRHLMYVIWQRTDSPEAFYACSDVDFDVALPLYSTT

SEQ ID NO: 205 - protein, 215 aa, Polypodium attenuatum (Falax)
MGKGWEVVGIMVVCACGLLGVASGHGTMEDPISRVYRCRLENPERPTSPACIAAVALSGTQAFYDWNEVNLPFAAGRHREIIPDGQLCSAGRAKYRGLDLARDDWLATSLSSGVDYTFVYRVTAPHRGYFEFYVTRDTYDPTEPLKWSDLEEPPFINVTQPSLVSGSYQIPGATPTGKTGRHLIYVIWQRTDSPEAFYSCSDVDFGEALRLDATA

SEQ ID NO: 206 - protein, 215 aa, Arachniodes simplicior (variegata)
MGRSWGVVAIIVLCASGLLGVASGHGSMEDPISRVYNCFLEGPENPTSDACIAAVALSGTQAFYDWTEVNLADADGHHRELIPDGQLCSAGRDKYKGLDLARSDWTATSLSSGVDYTFLFKATAPHLGSFEFYVTVDGYEPTEPLKWADLEATPFINVTDPTLDSGSYQIPGTTPAGKTGRHLIYVIWQRSDSAEAFYSCSDVDFTDALSLHSTT

SEQ ID NO: 207 - protein, 216 aa, Campyloneurum angustifolium
MRRSWEVVGMMVLCACGLLGVASGHGSMEDPISRVYRCRLEGPERPTSPACIAAVAVNGTQAFYDWNEVNQPFAAGRHREIIPDGQLCSAGRDKYKGLDLARADWLAVSLSSGADYTFLYLATATHRGYFEFYVTRDSYDPTEPLKWSDLEDSPFINVTDPTEVGPVYQIPGTTPAGKTGRHLIYVIWQRTDSPEAFYSCSDVDFGESLSLYSVTE

SEQ ID NO: 208 - protein, 215 aa, Colysis wrightii (Ching)
MRKSLEVVAIMVAVCASGLLGVASGHGTMLDPISRVYRCYLENPERPTSPACIAAVALSGKQAFYDWNEVNLPFAAGRHRELIPDGQLCSAGRDKYKGLDQARDDWLATSLPSGANYIFRFEVTAVHRGYFEFYVTRDGYDPTQPLAWADLEDSPFLTTTTTLDSSSYIIPGTTPAGKTGRHLIYLIWQRTDSPEAFYSCSDVDFEEAISLSSTT

SEQ ID NO: 209 - protein, 246 aa, Colysis wrightii (Ching)
MGRSWVVVAIMVTVCASGLLGFASGHGSMGDPISRVLRCREENPENPTSPACIAAVALSGKQAFYDWNEVNLPFAAGRHRELIPDGQLCSAGRAKYKGLDLARDDWLATPLPSGAAYTFRYRVTAAHRGYFEFYVTRDGYDPTQPLAWADLEDSPFLTTTTTLDSSSYIIPGTTPAGKTGRHLIYLIWQRTDSPEAFYSCSDVDFEEAISLSSTTLSLAGGLSGMATYCKGHAAAPVLTWRMECCC

SEQ ID NO: 210 - protein, 216 aa, Platycerium elephantotis
MRRSWGVVAVMLAICASGLLGVASGHGSMLDPISRVYTCYLENPERPTSAACIAAVAVSGSQAFYDWNEVNLADADGQHRQLIPDGKLCSAGREKYRGLDLARDDWPATSLSSGVNYTFLYRATAPHLGFFEFYVTRDSYDPTQPLAWADLEDPPFINITDPTLASGSYQIVNTTPSNKTGRHLIYVIWQRTDSPEAFYSCSDVDFDEDDSLLSAV

SEQ ID NO: 211 - protein, 215 aa, Platycerium madagascariense
MRRSWGVVAVILAMCAGSLLGVASGHGSMEDPISRVYACFLENPERPTSAACIAAVALSGTQAFYDWNEVNQPNAAGNHTIIPDGQLCSAGREKYKGLDLPRADWSAISLSSGVNYTFLYKATAPHRGYFEFYVTRDSYDPTEPLAWADLEDTPFINITDPDLVSGSYRIANTTPSGKTGRHLIYVIWQRTDSPEAFYSCSDVVFDEDVSLVSAA

SEQ ID NO: 212 - protein, 216 aa, Microsorum musifolium (Blume)
MRRSWGVLAIVVAVCASGLFGVASGHGSMEHPISRVYQCYREGPENPKSPACIAAKGLSGAQAFYDWNEVNQPFADGRHQEIIHDGHLCSGGRDKYRGLDLPRADWVATSLSAGKPYTFLYRATAPHLGYFQFYVTRDGYNPTKPLAWADLEDSPFINVTNPTLVSGSYRIPHTTPASKTGRHLIYVIWQRTDSPEAFYSCSDVVFDEALSLSSTI

SEQ ID NO: 213 - protein, 219 aa, Lygodium flexuosum
MGSWQWGSVNVAIVVFMMLCGVASGHGTMGDPISRVYRCYLENPERPTSAACQAAVALSGTQAFYDWNEVNLPNAAGRHRQLIPDGQLCSAGRAKYQGLDLARADWLAASLSSGVSYTFLYRVTAQHRGFFEFYVTRDGYEPTEPLKWSDLEESPFINVTDPTAVSGSYQIPGTTPAGKSGRHLIYVIWQRSDSPEAFYSCSDVDFDVEGAAVSLRSTT

SEQ ID NO: 214 - protein, 215 aa, Polystichum polyblepharum
MNRSWGVVAIMVLCASGLLGVASGHGTMNDPISRVYNCRLENPESPTSAACIAAVALSGTQAFYDWNEVNLANVAGRHRELIPDGKLCSAGRDKYKGLDLARSDWVATNLSSGVAFTFLYRVTAQHRGFFEFYVTVDDYDPTELLKWEDLEETPFMNVTDPTLVGLNYEMPGTTPANKTGRHLIYVIWQRSDSPEAFYSCSDVDFVDAVSLHSST

SEQ ID NO: 215 - protein, 218 aa, Diplazium pycnocarpon
MGKSWGVVAIILVLCASGLLGVASGHGSMADPISRIYNCRQENPERPTSAACQAAVALSGTQAFYDWNEVNQPNAAGRHREIIPDGQLCSAGRYKYRGLDLASADWQWPATSLSSGVSFTYRYRATAAHYGYFQFYITRDGYQPTQPLKWADLEQLPFLTVYNPTLVNGFYEMQGTTPAGKTGRHLIYVIWQRSDSPEAFYSCSDVDFVGALSLHSTT

SEQ ID NO: 216 - protein, 216 aa, Polystichum braunii
MGRSWGVVAIMVLCASGLLGAASGHGTMYDPFSRVYNCRFRENPERPTSAACIAAVALSGTQAFYDWNEVNLANAAGRHRELIPDGKLCSAGRDKYKGLDLARSDWVATNLSSGVAFTFLYRVTAQHRGFFEFYVTVDDYDPTESLKWEDLEETPFLNVTDPTVVGVNYQISGTTPASKTGRHLIYVIWQRSDSPEAFYSCSDVDFVDALSLQSTT

SEQ ID NO: 217 - protein, 215 aa, Platycerium hillii
MGKPWRVVVAIVVVCASGLLGVASGHGSMGEPISRVYNCYLENPERPTSAACIAAVALSGTQAFYDWNEVNLPFAAGRHRELIPDGQLCSAGRDKYKGLDLARADWVATSLSSGVSYTFLYRVTAPHRGYFEFYVTKDSYDPTEPLAWADLEDTPFINITDPTIVSGSYQISSTTPSDKTGRHLIYVIWQRTDSPEAFYSCSDIDFDDTLPLHST

SEQ ID NO: 218 - protein, 227 aa, Drynaria rigidula (whitei)
MGRTYSWGAVAVMVVLCASGLLGIASGHGSMDSPISRVYRCYLENPENPTSAACQAAVALSGTQAFYDWNEVNIADAAGRHRELIPDGQLCSAGREKYQGLDLARADWLADSLSSGVSFTFLYKATAAHLGFFEFYVTRDAYDPTEPLKWADLEDSPFLNVTDPTLVSGYYQIPGTTPAGKSGRHLLYVIWQRSDSPEAFYSCSDVDFDDDAAAAQHMIISLRHSTT

SEQ ID NO: 219 - protein, 229 aa, Adiantum monocolor; identical to SEQ ID NO: 165

SEQ ID NO: 220 - protein, 223 aa, Pellaea rotundifolia
MQRSCMWGESVVAIMCMVLGLLGDVASGHGSMASPISRVFNCYLENPESPTSEACKAAVEESGTQAFYDWAEVSLPNAAGRHRELIPDGQLCSAGLAKYAGLDLARADWTATSLTSNISYTFIFEATAGPHLGSFEFYVTNDDYEPAEALNWADLEDTPFIIVTNPTLVSGSYLIPGTTPAGKTGRHIIYVIWQRSDSPEAFYSCSDIDFVEEDPVVPLHSTT

SEQ ID NO: 221 - protein, 216 aa, Microsorum punctatum
MRRSWGVLAIVVAVCASGLFGVASGHGSMEDPISRVYQCYDEGPENPKSPACIAAVGLSGAQAFYDWNEVNQPFAAGQHKEIIHDGHLCSGGRDKYRGLDLPRADWVATSLSAGAPYTFLYRATAHHLGYFEFYVTRDGYDPTKPLAWADLEDSPFINVTNPPLVSGSYRIPDTTPALKTGRHLIYVIWQRTDSPEAFYSCSDVVFAEALSLSSTT

SEQ ID NO: 222 - protein, 217 aa, Woodwardia fimbriata
MGRSIWGVVAMMVLCASGLLRIASGHGSMENPISRVYNCYLEGPENPKSAACKAAVAASGTQAFYDWNEVNLANAAGRHRELIPDGQLCSAGRQKYQGLDLVRSDWPATSLSSGVPFTFLYRITAQHLGFFEFYVTRDGYQPTAALTWADLEDSPFMNVTGDPTFITGSWEIPGTSPAGKSGRHLIYVIWQRSDSPEAFYACCDVDFVDALSLHSTT

SEQ ID NO: 223 - protein, 213 aa, Dryopteris celsa
MGRSSLGVVAIMVLCLVGVASGHGSMQDPISRVYNCYLENPESPTSAACQAAVALSGTQAFYDWNEVNQPEADGRSREIIPDGQLCSGGREKYQGLDLARSDWEATTLSSSVNYTFLYKATAPHLGFFEFYVTQDGYDPTEVLKWADLEDSPFLNVTDPTLDSGAYQIPGTTPAGKTGRHLIYVIWQRSDSPEAFYSCSDVDFPDALSLHSTT

SEQ ID NO: 224 - protein, 216 aa, Campyloneurum angustifolium
MRRSWEVVGMMVLCACGLLGVASGHGSMEDPISRVYRCRLENPERPTSPACRAAVALSGTQAFYDWNEVNQPFAAGRHREIIPDGQLCSAGRDKYKGLDLARADWLAVSLSSGADYTFLYLATATHRGYFEFYVTRDSYDPTEPLKWSDLEDSPFINVTDPTEVGPVYQIPGTTPAGKTGRHLIYVIWQRTDSPEAFYSCSDVDFGESLSLYSVTE

SEQ ID NO: 225 - protein, 218 aa, Onoclea sensibilis
MGRSWGVVQAIIMVLCGSGLLGVASGHGSMEDPISRVYNCYLENPESPTSAACQAAVALSGAQAFYDWNEVNLADAAGRHRELIPDGQLCSAGREKYQGLDLARSDWTATSLSSGVSFTYLYKATAPHLGFFEFYVTKDGYEPTEPLKWADLEDSPLINVTDPTLVSGSYQIPGTTPSGKSGRHLIYVIWQRSDSPEAFYSCSDVDFDVDALSLHSTT

SEQ ID NO: 226 - protein, 235 aa, Onoclea sensibilis
MGRSWGVVQAIIMVLCGSGLLGVASGHGSMEDPISRVYNCYLENPESPTSAACQAAVALSGAQAFYDWNEVNLADAAGRHRELIPDGQLCSAGREKYQGLDLARSDWTATSLSSGVSFTYLYKATAPHLGFFEFYVTKDGYEPTEPLKWADLEDSPFINVTDPTLVSGSYQIPGTTPSGKSGRHLIYVIWQRSDSPEAFYSCSDVDFDVDALSLHSTPNLDLSSSGLANLINVCV

SEQ ID NO: 227 - protein, 229 aa, Onoclea sensibilis
MGRSWGVVQAIIMVLCGSGLLGVASGHGSMEDPISRVYNCYLENPESPTSAACQAAVALSGAQAFYDWNEVNLADAAGRHRELIPDGQLCSAGREKYQGLDLARSDWTATSLSSGVSFTYLYKATAPHLGFFEFYVTKDGYEPTEPLKWADLEDSPFINVTDPTLVSGSYQIPGTTPSGKSGRHLIYVIWQRSDSPEAFYSCSDVDFDVDALSLHSTPNLDLSILDWPT

SEQ ID NO: 228 - protein, 215 aa, Polystichum tripteron
MGRSWGVVAIMVLCASGLLGVASGHGTMNDPISRVYACRQENPERPTTPACIAAVALSGAQAFYDWNEVNLPFVNGRHRQFIPDGKLCSAGRNKYRGLDLARSDWTATNLSSGVAYTFLYRVTAQHRGFFEFYVTVDGYDPTEPLKWADLEETPFINVTDPTVVGLNYVIPGTTPASKTGRHLIYVIWQRSDSPEAFYSCSDVNFPDALSLHSAT

SEQ ID NO: 229 - protein, 215 aa, Polystichum tripteron
MGRSWGVVAIMVLCASGLLGVASGHGTMNDPISRVYACRQENPERPTTPACIAAVALSGAQAFYDWNEVNLPFVNGRHRQFIPDGKLCSAGRNKYRGLDLARSDWTATNLSSGVAYTFLYRVTAQHRGFFEFYVTVDGYDPTEPLKWADLEETPFINVTDPTVVGLNYVISGTTPASKTGRHLIYVIWQRTDSPEAFYSCSDVNFPDALSLHSAT

SEQ ID NO: 230 - protein, 215 aa, Polystichum tripteron
MGRSWGVVAIMMLCASGLLGVASGHGTMNDPISRVYACRQENPERPTTPACIAAVALSGAQAFYDWNEVNLPFVNGRHRQFIPDGKLCSAGRNKYRGLDLARSDWTATNLSSGVAYTFLYRVTAQHRGFFEFYVTVDGYDPTEPLKWADLEETPFINVTDPTVVGLNYVIPGTTPASKTGRHLIYVIWQRSDSPEAFYSCSDVNFPDALSLHSAT

SEQ ID NO: 231 - protein, 215 aa, Polystichum tripteron
MGRSWGVVAIMVLCASGLLGVASGHGTMNDPISRVYACRQENPERPTTPACIAAVALSGAQAFYDWNEVNLPFVNGRHRQFIPDGKLCSAGRNKYRGLDLARSDWTATNLSSGVAYTFLYRVTAQHRGFFEFYVTVDGYDPTEPLKWADLEETPFINVANPTVVGLNYVISGTTPASKTGRHLIYVIWQRTDSPEAFYSCSDVNFVDALSLHSAT

SEQ ID NO: 232 - protein, 217 aa, Tectaria milnei
MGRSWGVVAVMVVCASGLLSVVRGHGSMEDPISRVYACFLENPERPISAACQAAVAMGGTQAFYDWNAVSLPYAAGRHRELIPDGQLCSAGRAKYRGLDLPRDDWPGTSNMTSGVAFTYRYKATAPHLGSFQFYVTRDGYDPTEPLKWADLEDSPFMNATSTLAPDSYLMSGTTPSGKAGHHLIYAIWQRSDSPEAFYSCSDVTFDVAAVSDLHSTT

SEQ ID NO: 233 - protein, 217 aa, Tectaria milnei
MGRSWGVVAVMVVCASGLLSVVRGHGSMEDPISRVYACFLENPERPISAACQAAVAMGGTQAFYDWNAVSLPYAAGRHRELIPDGQLCSAGRAKYRGLDLPRDDWPGTSNMTSGVAFTYRYKATAPHLGSFQFHVTRDGYDPTEPLKWADLEDSPFMNATSTLAPDSYLMSGTTPSGKAGHHLIYAIWQRSDSPEAFYSCSDVTFDVAAVSDLHSTT

SEQ ID NO: 234 - protein, 217 aa, Tectaria milnei
MGRSWGVVAVMVVCASGLLSVVRGHGSMEDPISRVYACFLENPERPISAACQAAVAMGGTQAFYDWNAVSLPYAAGRHRELIPDGQLCSAGRAKYRGLDLPRDDWPGTSNMTSGVAFTYRYKATAPHLGSFQFYVTRDGYDPTEPLKWADLEDSPLMNATSTLAPDSYLMSGTTPSGKAGHHLIYAIWQRSDSPEAFYSCSDVTFDVAAVSDLHSTT

SEQ ID NO: 235 - DNA, 51 bp, Unknown
  Synthetic sequence
gtttaactttaagaaggagatatacatatgggcaggtcatggggagttgtg

SEQ ID NO: 236 - DNA, 49 bp, Unknown
  Synthetic sequence
gtgatggtgatggtgatggtgggatccggtggtggagtggagagatagg

SEQ ID NO: 237 - DNA, 49 bp, Unknown
  Synthetic sequence
gtttaactttaagaaggagatatacatatggggagatcatggggagttg

SEQ ID NO: 238 - DNA, 49 bp, Unknown
  Synthetic sequence
gtgatggtgatggtgatggtgggatccggtggtggagtggagagagagg

SEQ ID NO: 239 - DNA, 49 bp, Unknown
  Synthetic sequence
gtttaactttaagaaggagatatacatatggggaggtcatggggagttg

SEQ ID NO: 240 - DNA, 50 bp, Unknown
  Synthetic sequence
gtgatggtgatggtgatggtgggatccggtggtagagtggagagagagag

SEQ ID NO: 241 - DNA, 51 bp, Unknown
  Synthetic sequence
gtttaactttaagaaggagatatacatatggggaggccatggggagttgtg

SEQ ID NO: 242 - DNA, 49 bp, Unknown; identical to SEQ ID NO: 238
  Synthetic sequence

SEQ ID NO: 243 - DNA, 55 bp, Unknown
  Synthetic sequence
aatctctcatctaagaggctggatcctaggatggggaggtcatggggagtggtgc

SEQ ID NO: 244 - DNA, 55 bp, Unknown
  Synthetic sequence
tggccaatccagaagatggacaagtctagattaggtggtggagtggagagagagg

SEQ ID NO: 245 - DNA, 55 bp, Unknown
  Synthetic sequence
aatctctcatctaagaggctggatcctaggatggggaggtcatggggagtggtgg

SEQ ID NO: 246 - DNA, 55 bp, Unknown
  Synthetic sequence
tggccaatccagaagatggacaagtctagattaggtggtggagtggagatcagag

SEQ ID NO: 247 - DNA, 55 bp, Unknown
  Synthetic sequence
aatctctcatctaagaggctggatcctaggatgggcaggtcatggggagttgtgg

SEQ ID NO: 248 - DNA, 55 bp, Unknown
  Synthetic sequence
tggccaatccagaagatggacaagtctagattaggtggcggagtggagagacagg

SEQ ID NO: 249 - protein, 5 aa, Unknown
  Synthetic sequence
EEKKN